European Patent Application EP 4 344 705 A2, published April 3, 2024. Title: BIOMARKERS AND METHODS FOR PREDICTING PREECLAMPSIA. Applicant: SERA PROGNOSTICS, INC. Application EP. The sequence listing filed with the application follows.

SEQUENCE LISTING (964 sequences)

SEQ ID NO: 1 - protein, 7 aa, Homo sapiens
FSVVYAK

SEQ ID NO: 2 - protein, 9 aa, Homo sapiens
SPELQAEAK

SEQ ID NO: 3 - protein, 10 aa, Homo sapiens
VNHVTLSQPK

SEQ ID NO: 4 - protein, 19 aa, Homo sapiens
SSNNPHSPIVEEFQVPYNK

SEQ ID NO: 5 - protein, 9 aa, Homo sapiens
VVGGLVALR

SEQ ID NO: 6 - protein, 9 aa, Homo sapiens
LDFHFSSDR

SEQ ID NO: 7 - protein, 10 aa, Homo sapiens
TVQAVLTVPK

SEQ ID NO: 8 - protein, 7 aa, Homo sapiens
GPGEDFR

SEQ ID NO: 9 - protein, 8 aa, Homo sapiens
ETLLQDFR

SEQ ID NO: 10 - protein, 9 aa, Homo sapiens
ATVVYQGER

SEQ ID NO: 11 - protein, 12 aa, Homo sapiens
GFQALGDAADIR

SEQ ID NO: 12 - protein, 18 aa, Homo sapiens
SSNNPHSPIVEEFQVPYN

SEQ ID NO: 13 - protein, 11 aa, Homo sapiens
TSDQIHFFFAK

SEQ ID NO: 14 - protein, 11 aa, Homo sapiens
DPNGLPPEAQK

SEQ ID NO: 15 - protein, 13 aa, Homo sapiens
SVSLPSLDPASAK

SEQ ID NO: 16 - protein, 15 aa, Homo sapiens
IEGNLIFDPNNYLPK

SEQ ID NO: 17 - protein, 10 aa, Homo sapiens
YWGVASFLQK

SEQ ID NO: 18 - protein, 14 aa, Homo sapiens
ITENDIQIALDDAK

SEQ ID NO: 19 - protein, 11 aa, Homo sapiens
GWVTDGFSSLK

SEQ ID NO: 20 - protein, 10 aa, Homo sapiens
TGISPLALIK

SEQ ID NO: 21 - protein, 10 aa, Homo sapiens
IIGGSDADIK

SEQ ID NO: 22 - protein, 10 aa, Homo sapiens
TLLIANETLR

SEQ ID NO: 23 - protein, 15 aa, Homo sapiens
VSALLTPAEQTGTWK

SEQ ID NO: 24 - protein, 16 aa, Homo sapiens
DALSSVQESQVAQQAR

SEQ ID NO: 25 - protein, 9 aa, Homo sapiens
IAQYYYTFK

SEQ ID NO: 26 - protein, 7 aa, Homo sapiens
IEEIAAK

SEQ ID NO: 27 - protein, 22 aa, Homo sapiens
VILGAHQEVNLEPHVQEIEVSR

SEQ ID NO: 28 - protein, 7 aa, Homo sapiens
DYWSTVK

SEQ ID NO: 29 - protein, 10 aa, Homo sapiens
VPLALFALNR

SEQ ID NO: 30 - protein, 9 aa, Homo sapiens
VIAVNEVGR

SEQ ID NO: 31 - protein, 8 aa, Homo sapiens
LLEVPEGR

SEQ ID NO: 32 - protein, 20 aa, Homo sapiens
VEPLYELVTATDFAYSSTVR

SEQ ID NO: 33 - protein, 9 aa, Homo sapiens
HHGPTITAK

SEQ ID NO: 34 - protein, 24 aa, Homo sapiens
ALNFGGIGVVVGHELTHAFDDQGR

SEQ ID NO: 35 - protein, 14 aa, Homo sapiens
GGEGTGYFVDFSVR

SEQ ID NO: 36 - protein, 16 aa, Homo sapiens
SPEQQETVLDGNLIIR

SEQ ID NO: 37 - protein, 11 aa, Homo sapiens
EPGLCTWQSLR

SEQ ID NO: 38 - protein, 24 aa, Homo sapiens
VVLSSGSGPGLDLPLVLGLPLQLK

SEQ ID NO: 39 - protein, 7 aa, Homo sapiens
YTTEIIK

SEQ ID NO: 40 - protein, 12 aa, Homo sapiens
EDTPNSVWEPAK

SEQ ID NO: 41 - protein, 18 aa, Homo sapiens
LHEAFSPVSYQHDLALLR

SEQ ID NO: 42 - protein, 6 aa, Homo sapiens
AHYDLR

SEQ ID NO: 43 - protein, 16 aa, Homo sapiens
GDTYPAELYITGSILR

SEQ ID NO: 44 - protein, 22 aa, Homo sapiens
TSESGELHGLTTEEEFVEGIYK

SEQ ID NO: 45 - protein, 11 aa, Homo sapiens
ALEQDLPVNIK

SEQ ID NO: 46 - protein, 9 aa, Homo sapiens
LPNNVLQEK

SEQ ID NO: 47 - protein, 7 aa, Homo sapiens
FQLPGQK

SEQ ID NO: 48 - protein, 10 aa, Homo sapiens
HTLNQIDEVK

SEQ ID NO: 49 - protein, 10 aa, Homo sapiens
DADPDTFFAK

SEQ ID NO: 50 - protein, 7 aa, Homo sapiens
HFQNLGK

SEQ ID NO: 51 - protein, 18 aa, Homo sapiens
FNAVLTNPQGDYDTSTGK

SEQ ID NO: 52 - protein, 16 aa, Homo sapiens
ALNHLPLEYNSALYSR

SEQ ID NO: 53 - protein, 6 aa, Homo sapiens
AWVAWR

SEQ ID NO: 54 - protein, 12 aa, Homo sapiens
ETAASLLQAGYK

SEQ ID NO: 55 - protein, 14 aa, Homo sapiens
IALGGLLFPASNLR

SEQ ID NO: 56 - protein, 16 aa, Homo sapiens
IAPQLSTEELVSLGEK

SEQ ID NO: 57 - protein, 18 aa, Homo sapiens
VAPEEHPVLLTEAPLNPK

SEQ ID NO: 58 - protein, 15 aa, Homo sapiens
IPGIFELGISSQSDR

SEQ ID NO: 59 - protein, 9 aa, Homo sapiens
IQTHSTTYR

SEQ ID NO: 60 - protein, 10 aa, Homo sapiens
LLDSLPSDTR

SEQ ID NO: 61 - protein, 19 aa, Homo sapiens
QLGLPGPPDVPDHAAYHPF

SEQ ID NO: 62 - protein, 16 aa, Homo sapiens
SYELPDGQVITIGNER

SEQ ID NO: 63 - protein, 7 aa, Homo sapiens
WGAAPYR

SEQ ID NO: 64 - protein, 14 aa, Homo sapiens
DFHINLFQVLPWLK

SEQ ID NO: 65 - protein, 22 aa, Homo sapiens
VPTADLEDVLPLAEDITNILSK

SEQ ID NO: 66 - protein, 11 aa, Homo sapiens
LIENGYFHPVK

SEQ ID NO: 67 - protein, 17 aa, Homo sapiens
NKPGVYTDVAYYLAWIR

SEQ ID NO: 68 - protein, 11 aa, Homo sapiens
NTVISVNPSTK

SEQ ID NO: 69 - protein, 7 aa, Homo sapiens
LPDATPK

SEQ ID NO: 70 - protein, 14 aa, Homo sapiens
LEQGENVFLQATDK

SEQ ID NO: 71 - protein, 8 aa, Homo sapiens
TLYSSSPR

SEQ ID NO: 72 - protein, 20 aa, Homo sapiens
DGSPDVTTADIGANTPDATK

SEQ ID NO: 73 - protein, 15 aa, Homo sapiens
EWVAIESDSVQPVPR

SEQ ID NO: 74 - protein, 8 aa, Homo sapiens
LYYGDDEK

SEQ ID NO: 75 - protein, 24 aa, Homo sapiens
ADSQAQLLLSTVVGVFTAPGLHLK

SEQ ID NO: 76 - protein, 7 aa, Homo sapiens
AYSDLSR

SEQ ID NO: 77 - protein, 10 aa, Homo sapiens
DLHLSDVFLK

SEQ ID NO: 78 - protein, 10 aa, Homo sapiens
LSSPAVITDK

SEQ ID NO: 79 - protein, 8 aa, Homo sapiens
SGFSFGFK

SEQ ID NO: 80 - protein, 16 aa, Homo sapiens
IIEVEEEQEDPYLNDR

SEQ ID NO: 81 - protein, 8 aa, Homo sapiens
AVYEAVLR

SEQ ID NO: 82 - protein, 22 aa, Homo sapiens
FTFTLHLETPKPSISSSNLNPR

SEQ ID NO: 83 - protein, 10 aa, Homo sapiens
DAQYAPGYDK

SEQ ID NO: 84 - protein, 11 aa, Homo sapiens
YGLVTYATYPK

SEQ ID NO: 85 - protein, 9 aa, Homo sapiens
DISEVVTPR

SEQ ID NO: 86 - protein, 13 aa, Homo sapiens
IVLGQEQDSYGGK

SEQ ID NO: 87 - protein, 9 aa, Homo sapiens
TLEAQLTPR

SEQ ID NO: 88 - protein, 22 aa, Homo sapiens
VPVAVQGEDTVQSLTQGDGVAK

SEQ ID NO: 89 - protein, 13 aa, Homo sapiens
AEAQAQYSAAVAK

SEQ ID NO: 90 - protein, 10 aa, Homo sapiens
ELLESYIDGR

SEQ ID NO: 91 - protein, 11 aa, Homo sapiens
TNLESILSYPK

SEQ ID NO: 92 - protein, 9 aa, Homo sapiens
LPTAVVPLR

SEQ ID NO: 93 - protein, 14 aa, Homo sapiens
DSPVLIDFFEDTER

SEQ ID NO: 94 - protein, 7 aa, Homo sapiens
FAFNLYR

SEQ ID NO: 95 - protein, 12 aa, Homo sapiens
FVFGTTPEDILR

SEQ ID NO: 96 - protein, 15 aa, Homo sapiens
GDSGGAFAVQDPNDK

SEQ ID NO: 97 - protein, 13 aa, Homo sapiens
SLDFTELDVAAEK

SEQ ID NO: 98 - protein, 7 aa, Homo sapiens
SLLQPNK

SEQ ID NO: 99 - protein, 16 aa, Homo sapiens
VQEAHLTEDQIFYFPK

SEQ ID NO: 100 - protein, 11 aa, Homo sapiens
DDLYVSDAFHK

SEQ ID NO: 101 - protein, 22 aa, Homo sapiens
DPDQTDGLGLSYLSSHIANVER

SEQ ID NO: 102 - protein, 10 aa, Homo sapiens
ESDTSYVSLK

SEQ ID NO: 103 - protein, 8 aa, Homo sapiens
ILDDLSPR

SEQ ID NO: 104 - protein, 15 aa, Homo sapiens
SLPVSDSVLSGFEQR

SEQ ID NO: 105 - protein, 16 aa, Homo sapiens
TWDPEGVIFYGDTNPK

SEQ ID NO: 106 - protein, 10 aa, Homo sapiens
VGEYSLYIGR

SEQ ID NO: 107 - protein, 15 aa, Homo sapiens
VPGTSTSATLTGLTR

SEQ ID NO: 108 - protein, 15 aa, Homo sapiens
YEVQGEVFTKPQLWP

SEQ ID NO: 109 - protein, 13 aa, Homo sapiens
AFTECCVVASQLR

SEQ ID NO: 110 - protein, 8 aa, Homo sapiens
APLTKPLK

SEQ ID NO: 111 - protein, 8 aa, Homo sapiens
FLQEQGHR

SEQ ID NO: 112 - protein, 14 aa, Homo sapiens
ISLLLIESWLEPVR

SEQ ID NO: 113 - protein, 10 aa, Homo sapiens
LQGTLPVEAR

SEQ ID NO: 114 - protein, 14 aa, Homo sapiens
SYTITGLQPGTDYK

SEQ ID NO: 115 - protein, 8 aa, Homo sapiens
TASDFITK

SEQ ID NO: 116 - protein, 17 aa, Homo sapiens
VLSALQAVQGLLVAQGR

SEQ ID NO: 117 - protein, 8 aa, Homo sapiens
VTGWGNLK

SEQ ID NO: 118 - protein, 12 aa, Homo sapiens
AFIQLWAFDAVK

SEQ ID NO: 119 - protein, 11 aa, Homo sapiens
GYVIIKPLVWV

SEQ ID NO: 120 - protein, 18 aa, Homo sapiens
IITGLLEFEVYLEYLQNR

SEQ ID NO: 121 - protein, 13 aa, Homo sapiens
TDAPDLPEENQAR

SEQ ID NO: 122 - protein, 8 aa, Homo sapiens
TFTLLDPK

SEQ ID NO: 123 - protein, 7 aa, Homo sapiens
VLEPTLK

SEQ ID NO: 124 - protein, 7 aa, Homo sapiens
YEFLNGR

SEQ ID NO: 125 - protein, 23 aa, Homo sapiens
AITPPHPASQANIIFDITEGNLR

SEQ ID NO: 126 - protein, 12 aa, Homo sapiens
RIVQIYKDLLRN

SEQ ID NO: 127 - protein, 10 aa, Homo sapiens
KVMNHICSKQ

SEQ ID NO: 128 - protein, 14 aa, Homo sapiens
RRHPDLSIPELLRI

SEQ ID NO: 129 - protein, 9 aa, Homo sapiens
KHFQNLGKD

SEQ ID NO: 130 - protein, 13 aa, Homo sapiens
KITLLSALVETRT

SEQ ID NO: 131 - protein, 20 aa, Homo sapiens
RLYGSEAFATDFQDSAAAKK

SEQ ID NO: 132 - protein, 12 aa, Homo sapiens
RNLAVSQVVHKA

SEQ ID NO: 133 - protein, 16 aa, Homo sapiens
RCEGPIPDVTFELLRE

SEQ ID NO: 134 - protein, 39 aa, Homo sapiens
RLHDNQNGWSGDSAPVELILSDETLPAPEFSPEPESGRA

SEQ ID NO: 135 - protein, 24 aa, Homo sapiens
RTPGAAANLELIFVGPQHAGNYRC

SEQ ID NO: 136 - protein, 10 aa, Homo sapiens
KLLELTGPKS

SEQ ID NO: 137 - protein, 13 aa, Homo sapiens
RATWSGAVLAGRD

SEQ ID NO: 138 - protein, 26 aa, Homo sapiens
KHQMDLVATLSQLGLQELFQAPDLRG

SEQ ID NO: 139 - protein, 15 aa, Homo sapiens
KLGNQEPGGQTALKS

SEQ ID NO: 140 - protein, 28 aa, Homo sapiens
KGFPIKEDFLEQSEQLFGAKPVSLTGKQ

SEQ ID NO: 141 - protein, 31 aa, Homo sapiens
RQPNCDDPETEEAALVAIDYINQNLPWGYKH

SEQ ID NO: 142 - protein, 34 aa, Homo sapiens
KVWPQQPSGELFEIEIDTLETTCHVLDPTPVARC

SEQ ID NO: 143 - protein, 16 aa, Homo sapiens
KEHAVEGDCDFQLLKL

SEQ ID NO: 144 - protein, 12 aa, Homo sapiens
KHTLNQIDEVKV

SEQ ID NO: 145 - protein, 23 aa, Homo sapiens
RTVVQPSVGAAAGPVVPPCPGRI

SEQ ID NO: 146 - protein, 27 aa, Homo sapiens
KTGCSLMGASVDSTLAFNTYVHFQGKM

SEQ ID NO: 147 - protein, 16 aa, Homo sapiens
RAAMVGMLANFLGFRI

SEQ ID NO: 148 - protein, 19 aa, Homo sapiens
KQPFVQGLALYTPVVLPRS

SEQ ID NO: 149 - protein, 19 aa, Homo sapiens
KVLSALQAVQGLLVAQGRA

SEQ ID NO: 150 - protein, 26 aa, Homo sapiens
RADSQAQLLLSTVVGVFTAPGLHLKQ

SEQ ID NO: 151 - protein, 27 aa, Homo sapiens
RITDVIPSEAINELTVLVLVNTIYFKG

SEQ ID NO: 152 - protein, 23 aa, Homo sapiens
KNDNDNIFLSPLSISTAFAMTKL

SEQ ID NO: 153 - protein, 14 aa, Homo sapiens
REVPLNTIIFMGRV

SEQ ID NO: 154 - protein, 30 aa, Homo sapiens
RVAEGTQVLELPFKGDDITMVLILPKPEKS

SEQ ID NO: 155 - protein, 18 aa, Homo sapiens
KEQLQDMGLVDLFSPEKS

SEQ ID NO: 156 - protein, 13 aa, Homo sapiens
RDIPMNPMCIYRS

SEQ ID NO: 157 - protein, 22 aa, Homo sapiens
KEPCVESLVSQYFQTVTDYGKD

SEQ ID NO: 158 - protein, 19 aa, Homo sapiens
KSLAELGGHLDQQVEEFRR

SEQ ID NO: 159 - protein, 11 aa, Homo sapiens
RLAPLAEDVRG

SEQ ID NO: 160 - protein, 23 aa, Homo sapiens
RVLRENADSLQASLRPHADELKA

SEQ ID NO: 161 - protein, 27 aa, Homo sapiens
RSLAPYAQDTQEKLNHQLEGLTFQMKK

SEQ ID NO: 162 - protein, 19 aa, Homo sapiens
KLGPHAGDVEGHLSFLEKD

SEQ ID NO: 163 - protein, 29 aa, Homo sapiens
KSELTQQLNALFQDKLGEVNTYAGDLQKK

SEQ ID NO: 164 - protein, 13 aa, Homo sapiens
RLLPHANEVSQKI

SEQ ID NO: 165 - protein, 20 aa, Homo sapiens
KSLAELGGHLDQQVEEFRRR

SEQ ID NO: 166 - protein, 16 aa, Homo sapiens
KSELTQQLNALFQDKL

SEQ ID NO: 167 - protein, 14 aa, Homo sapiens
KGFEPTLEALFGKQ

SEQ ID NO: 168 - protein, 17 aa, Homo sapiens
KALYWVNGQVPDGVSKV

SEQ ID NO: 169 - protein, 9 aa, Homo sapiens
KFIIPSPKR

SEQ ID NO: 170 - protein, 9 aa, Homo sapiens
RTPALHFKS

SEQ ID NO: 171 - protein, 13 aa, Homo sapiens
KTEVIPPLIENRQ

SEQ ID NO: 172 - protein, 17 aa, Homo sapiens
RNLQNNAEWVYQGAIRQ

SEQ ID NO: 173 - protein, 18 aa, Homo sapiens
KLPQQANDYLNSFNWERQ

SEQ ID NO: 174 - protein, 11 aa, Homo sapiens
RLAAYLMLMRS

SEQ ID NO: 175 - protein, 19 aa, Homo sapiens
RVIGNMGQTMEQLTPELKS

SEQ ID NO: 176 - protein, 13 aa, Homo sapiens
KLIVAMSSWLQKA

SEQ ID NO: 177 - protein, 17 aa, Homo sapiens
RTSSFALNLPTLPEVKF

SEQ ID NO: 178 - protein, 24 aa, Homo sapiens
KIADFELPTIIVPEQTIEIPSIKF

SEQ ID NO: 179 - protein, 17 aa, Homo sapiens
KIEGNLIFDPNNYLPKE

SEQ ID NO: 180 - protein, 26 aa, Homo sapiens
RTSSFALNLPTLPEVKFPEVDVLTKY

SEQ ID NO: 181 - protein, 26 aa, Homo sapiens
RLELELRPTGEIEQYSVSATYELQRE

SEQ ID NO: 182 - protein, 23 aa, Homo sapiens
KSTAAMSTYTGIFTDQVLSVLKG

SEQ ID NO: 183 - protein, 22 aa, Homo sapiens
RGWVTDGFSSLKDYWSTVKDKF

SEQ ID NO: 184 - protein, 9 aa, Homo sapiens
RWELALGRF

SEQ ID NO: 185 - protein, 11 aa, Homo sapiens
RLAVYQAGARE

SEQ ID NO: 186 - protein, 14 aa, Homo sapiens
KSWFEPLVEDMQRQ

SEQ ID NO: 187 - protein, 17 aa, Homo sapiens
RAATVGSLAGQPLQERA

SEQ ID NO: 188 - protein, 18 aa, Homo sapiens
RTPEYYPNAGLIMNYCRN

SEQ ID NO: 189 - protein, 22 aa, Homo sapiens
KTFYEPGEEITYSCKPGYVSRG

SEQ ID NO: 190 - protein, 17 aa, Homo sapiens
KFICPLTGLWPINTLKC

SEQ ID NO: 191 - protein, 15 aa, Homo sapiens
RSLQTFSQAWFTCRR

SEQ ID NO: 192 - protein, 23 aa, Homo sapiens
KHYYIGIIETTWDYASDHGEKKL

SEQ ID NO: 193 - protein, 13 aa, Homo sapiens
REYTDASFTNRKE

SEQ ID NO: 194 - protein, 23 aa, Homo sapiens
KMYYSAVDPTKDIFTGLIGPMKI

SEQ ID NO: 195 - protein, 39 aa, Homo sapiens
RSGAGTEDSACIPWAYYSTVDQVKDLYSGLIGPLIVCRR

SEQ ID NO: 196 - protein, 25 aa, Homo sapiens
RKAEEEHLGILGPQLHADVGDKVKI

SEQ ID NO: 197 - protein, 16 aa, Homo sapiens
KEVGPTNADPVCLAKM

SEQ ID NO: 198 - protein, 24 aa, Homo sapiens
RMYSVNGYTFGSLPGLSMCAEDRV

SEQ ID NO: 199 - protein, 16 aa, Homo sapiens
KDIASGLIGPLIICKK

SEQ ID NO: 200 - protein, 30 aa, Homo sapiens
RQKDVDKEFYLFPTVFDENESLLLEDNIRM

SEQ ID NO: 201 - protein, 25 aa, Homo sapiens
RGPEEEHLGILGPVIWAEVGDTIRV

SEQ ID NO: 202 - protein, 15 aa, Homo sapiens
KGAYPLSIEPIGVRF

SEQ ID NO: 203 - protein, 25 aa, Homo sapiens
RGVYSSDVFDIFPGTYQTLEMFPRT

SEQ ID NO: 204 - protein, 17 aa, Homo sapiens
KDIASGLIGPLIICKKD

SEQ ID NO: 205 - protein, 25 aa, Homo sapiens
RSGAGTEDSACIPWAYYSTVDQVKD

SEQ ID NO: 206 - protein, 12 aa, Homo sapiens
RIYHSHIDAPKD

SEQ ID NO: 207 - protein, 35 aa, Homo sapiens
RADDKVYPGEQYTYMLLATEEQSPGEGDGNCVTRI

SEQ ID NO: 208 - protein, 16 aa, Homo sapiens
KDLYSGLIGPLIVCRR

SEQ ID NO: 209 - protein, 19 aa, Homo sapiens
RTTIEKPVWLGFLGPIIKA

SEQ ID NO: 210 - protein, 13 aa, Homo sapiens
KIFFPGVSEFGKE

SEQ ID NO: 211 - protein, 23 aa, Homo sapiens
RAILQSGSFNAPWAVTSLYEARN

SEQ ID NO: 212 - protein, 20 aa, Homo sapiens
RLHEAFSPVSYQHDLALLRL

SEQ ID NO: 213 - protein, 18 aa, Homo sapiens
RGDTYPAELYITGSILRM

SEQ ID NO: 214 - protein, 14 aa, Homo sapiens
KVLHGDLIDFVCKQ

SEQ ID NO: 215 - protein, 22 aa, Homo sapiens
KLVFQQFDLEPSEGCFYDYVKI

SEQ ID NO: 216 - protein, 12 aa, Homo sapiens
RVKNYVDWIMKT

SEQ ID NO: 217 - protein, 18 aa, Homo sapiens
KSNALDIIFQTDLTGQKK

SEQ ID NO: 218 - protein, 10 aa, Homo sapiens
RDFHINLFRM

SEQ ID NO: 219 - protein, 19 aa, Homo sapiens
RGALISDQWVLTAAHCFRD

SEQ ID NO: 220 - protein, 19 aa, Homo sapiens
KKNQGILEFYGDDIALLKL

SEQ ID NO: 221 - protein, 12 aa, Homo sapiens
RIHWESASLLRS

SEQ ID NO: 222 - protein, 11 aa, Homo sapiens
RVHYTVCIWRN

SEQ ID NO: 223 - protein, 15 aa, Homo sapiens
KAEMADQAAAWLTRQ

SEQ ID NO: 224 - protein, 21 aa, Homo sapiens
KMRPSTDTITVMVENSHGLRV

SEQ ID NO: 225 - protein, 24 aa, Homo sapiens
RVQQPDCREPFLSCCQFAESLRKK

SEQ ID NO: 226 - protein, 14 aa, Homo sapiens
KLVNGQSHISLSKA

SEQ ID NO: 227 - protein, 13 aa, Homo sapiens
RGQIVFMNREPKR

SEQ ID NO: 228 - protein, 23 aa, Homo sapiens
KVGLSGMAIADVTLLSGFHALRA

SEQ ID NO: 229 - protein, 19 aa, Homo sapiens
RGHLFLQTDQPIYNPGQRV

SEQ ID NO: 230 - protein, 11 aa, Homo sapiens
KSHALQLNNRQ

SEQ ID NO: 231 - protein, 25 aa, Homo sapiens
RYVSHFETEGPHVLLYFDSVPTSRE

SEQ ID NO: 232 - protein, 14 aa, Homo sapiens
RGSSTWLTAFVLKV

SEQ ID NO: 233 - protein, 16 aa, Homo sapiens
RYIYGKPVQGVAYVRF

SEQ ID NO: 234 - protein, 11 aa, Homo sapiens
KSCGLHQLLRG

SEQ ID NO: 235 - protein, 16 aa, Homo sapiens
RGPEVQLVAHSPWLKD

SEQ ID NO: 236 - protein, 29 aa, Homo sapiens
RKKEVYMPSSIFQDDFVIPDISEPGTWKI

SEQ ID NO: 237 - protein, 23 aa, Homo sapiens
RVQQPDCREPFLSCCQFAESLRK

SEQ ID NO: 238 - protein, 24 aa, Homo sapiens
KASAGLLGAHAAAITAYALTLTKA

SEQ ID NO: 239 - protein, 13 aa, Homo sapiens
KITHYNYLILSKG

SEQ ID NO: 240 - protein, 12 aa, Homo sapiens
RKAFDICPLVKI

SEQ ID NO: 241 - protein, 10 aa, Homo sapiens
RIPLDLVPKT

SEQ ID NO: 242 - protein, 28 aa, Homo sapiens
RMVETTAYALLTSLNLKDINYVNPVIKW

SEQ ID NO: 243 - protein, 17 aa, Homo sapiens
KALLVGEHLNIIVTPKS

SEQ ID NO: 244 - protein, 14 aa, Homo sapiens
KLKEGMLSIMSYRN

SEQ ID NO: 245 - protein, 18 aa, Homo sapiens
RYIYPLDSLTWIEYWPRD

SEQ ID NO: 246 - protein, 16 aa, Homo sapiens
KGGSASTWLTAFALRV

SEQ ID NO: 247 - protein, 28 aa, Homo sapiens
RYGGGFYSTQDTINAIEGLTEYSLLVKQ

SEQ ID NO: 248 - protein, 14 aa, Homo sapiens
KAKDLHLSDVFLKA

SEQ ID NO: 249 - protein, 18 aa, Homo sapiens
KALNHLPLEYNSALYSRI

SEQ ID NO: 250 - protein, 15 aa, Homo sapiens
RLSGNVLSYTFQVKI

SEQ ID NO: 251 - protein, 30 aa, Homo sapiens
RKDDIMLDEGMLQSLMELPDQYNYGMYAKF

SEQ ID NO: 252 - protein, 26 aa, Homo sapiens
RDFGTHYITEAVLGGIYEYTLVMNKE

SEQ ID NO: 253 - protein, 14 aa, Homo sapiens
RDTMVEDLVVLVRG

SEQ ID NO: 254 - protein, 17 aa, Homo sapiens
RYYAGGCSPHYILNTRF

SEQ ID NO: 255 - protein, 17 aa, Homo sapiens
RSLPVSDSVLSGFEQRV

SEQ ID NO: 256 - protein, 18 aa, Homo sapiens
RVQEAHLTEDQIFYFPKY

SEQ ID NO: 257 - protein, 31 aa, Homo sapiens
RTAGYGINILGMDPLSTPFDNEFYNGLCNRD

SEQ ID NO: 258 - protein, 15 aa, Homo sapiens
RRPWNVASLIYETKG

SEQ ID NO: 259 - protein, 15 aa, Homo sapiens
RAIEDYINEFSVRKC

SEQ ID NO: 260 - protein, 14 aa, Homo sapiens
RAIEDYINEFSVRK

SEQ ID NO: 261 - protein, 13 aa, Homo sapiens
RLEDSVTYHCSRG

SEQ ID NO: 262 - protein, 18 aa, Homo sapiens
RFIQVGVISWGVVDVCKN

SEQ ID NO: 263 - protein, 16 aa, Homo sapiens
RDFHINLFQVLPWLKE

SEQ ID NO: 264 - protein, 20 aa, Homo sapiens
KYGQTIRPICLPCTEGTTRA

SEQ ID NO: 265 - protein, 26 aa, Homo sapiens
RLLQEGQALEYVCPSGFYPYPVQTRT

SEQ ID NO: 266 - protein, 12 aa, Homo sapiens
RRPYFPVAVGKY

SEQ ID NO: 267 - protein, 13 aa, Homo sapiens
KCTSTGWIPAPRC

SEQ ID NO: 268 - protein, 11 aa, Homo sapiens
KCLHPCVISRE

SEQ ID NO: 269 - protein, 13 aa, Homo sapiens
REIMENYNIALRW

SEQ ID NO: 270 - protein, 20 aa, Homo sapiens
KAVYTCNEGYQLLGEINYRE

SEQ ID NO: 271 - protein, 22 aa, Homo sapiens
RSITCIHGVWTQLPQCVAIDKL

SEQ ID NO: 272 - protein, 12 aa, Homo sapiens
RWQSIPLCVEKI

SEQ ID NO: 273 - protein, 20 aa, Homo sapiens
KTDCLSLPSFENAIPMGEKK

SEQ ID NO: 274 - protein, 16 aa, Homo sapiens
KCFEGFGIDGPAIAKC

SEQ ID NO: 275 - protein, 11 aa, Homo sapiens
KIDVHLVPDRK

SEQ ID NO: 276 - protein, 14 aa, Homo sapiens
KSSNLIILEEHLKN

SEQ ID NO: 277 - protein, 15 aa, Homo sapiens
RAQLGDLPWQVAIKD

SEQ ID NO: 278 - protein, 12 aa, Homo sapiens
RVFSLQWGEVKL

SEQ ID NO: 279 - protein, 18 aa, Homo sapiens
RWSAGLTSSQVDLYIPKV

SEQ ID NO: 280 - protein, 22 aa, Homo sapiens
KTFPGFFSPMLGEFVSETESRG

SEQ ID NO: 281 - protein, 32 aa, Homo sapiens
RIEGSNKVPVDPATYGQFYGGDSYIILYNYRH

SEQ ID NO: 282 - protein, 24 aa, Homo sapiens
RAQPVQVAEGSEPDGFWEALGGKA

SEQ ID NO: 283 - protein, 28 aa, Homo sapiens
KTPSAAYLWVGTGASEAEKTGAQELLRV

SEQ ID NO: 284 - protein, 29 aa, Homo sapiens
RVEKFDLVPVPTNLYGDFFTGDAYVILKT

SEQ ID NO: 285 - protein, 17 aa, Homo sapiens
REVQGFESATFLGYFKS

SEQ ID NO: 286 - protein, 27 aa, Homo sapiens
KNWRDPDQTDGLGLSYLSSHIANVERV

SEQ ID NO: 287 - protein, 20 aa, Homo sapiens
KTPSAAYLWVGTGASEAEKT

SEQ ID NO: 288 - protein, 14 aa, Homo sapiens
KFLVGPDGIPIMRW

SEQ ID NO: 289 - protein, 29 aa, Homo sapiens
RLEKEVGTPHGIILDSVDAAFICPGSSRL

SEQ ID NO: 290 - protein, 15 aa, Homo sapiens
RWKNFPSPVDAAFRQ

SEQ ID NO: 291 - protein, 29 aa, Homo sapiens
RGECQAEGVLFFQGDREWFWDLATGTMKE

SEQ ID NO: 292 - protein, 26 aa, Homo sapiens
KEVGTPHGIILDSVDAAFICPGSSRL

SEQ ID NO: 293 - protein, 9 aa, Homo sapiens
RLWWLDLKS

SEQ ID NO: 294 - protein, 13 aa, Homo sapiens
KNFPSPVDAAFRQ

SEQ ID NO: 295 - protein, 14 aa, Homo sapiens
REWFWDLATGTMKE

SEQ ID NO: 296 - protein, 13 aa, Homo sapiens
KGGYTLVSGYPKR

SEQ ID NO: 297 - protein, 17 aa, Homo sapiens
KLYLVQGTQVYVFLTKG

SEQ ID NO: 298 - protein, 22 aa, Homo sapiens
REYYFAEAQIADFSDPAFISKT

SEQ ID NO: 299 - protein, 11 aa, Homo sapiens
KQFPILLDFKT

SEQ ID NO: 300 - protein, 9 aa, Homo sapiens
KFAFNLYRV

SEQ ID NO: 301 - protein, 11 aa, Homo sapiens
RDGYLFQLLRI

SEQ ID NO: 302 - protein, 24 aa, Homo sapiens
RSFEGLGQLEVLTLDHNQLQEVKA

SEQ ID NO: 303 - protein, 13 aa, Homo sapiens
RTFTPQPPGLERL

SEQ ID NO: 304 - protein, 12 aa, Homo sapiens
RAFWLDVSHNRL

SEQ ID NO: 305 - protein, 16 aa, Homo sapiens
RLAELPADALGPLQRA

SEQ ID NO: 306 - protein, 16 aa, Homo sapiens
RLEALPNSLLAPLGRL

SEQ ID NO: 307 - protein, 17 aa, Homo sapiens
RNLIAAVAPGAFLGLKA

SEQ ID NO: 308 - protein, 15 aa, Homo sapiens
RQAVDTAVDGVFIRS

SEQ ID NO: 309 - protein, 23 aa, Homo sapiens
KTAFISDFAVTADGNAFIGDIKD

SEQ ID NO: 310 - protein, 12 aa, Homo sapiens
RGHMLENHVERL

SEQ ID NO: 311 - protein, 30 aa, Homo sapiens
KTAFISDFAVTADGNAFIGDIKDKVTAWKQ

SEQ ID NO: 312 - protein, 39 aa, Homo sapiens
RGIEILNQVQESLPELSNHASILIMLTDGDPTEGVTDRS

SEQ ID NO: 313 - protein, 21 aa, Homo sapiens
KILGDMQPGDYFDLVLFGTRV

SEQ ID NO: 314 - protein, 12 aa, Homo sapiens
KLDAQASFLPKE

SEQ ID NO: 315 - protein, 18 aa, Homo sapiens
RGFSLDEATNLNGGLLRG

SEQ ID NO: 316 - protein, 25 aa, Homo sapiens
KTAFISDFAVTADGNAFIGDIKDKV

SEQ ID NO: 317 - protein, 21 aa, Homo sapiens
KGSLVQASEANLQAAQDFVRG

SEQ ID NO: 318 - protein, 15 aa, Homo sapiens
RLWAYLTIQELLAKR

SEQ ID NO: 319 - protein, 12 aa, Homo sapiens
REVAFDLEIPKT

SEQ ID NO: 320 - protein, 30 aa, Homo sapiens
RSILQMSLDHHIVTPLTSLVIENEAGDERM

SEQ ID NO: 321 - protein, 27 aa, Homo sapiens
KAGELEVFNGYFVHFFAPDNLDPIPKN

SEQ ID NO: 322 - protein, 17 aa, Homo sapiens
RETAVDGELVVLYDVKR

SEQ ID NO: 323 - protein, 35 aa, Homo sapiens
RNVQFNYPHTSVTDVTQNNFHNYFGGSEIVVAGKF

SEQ ID NO: 324 - protein, 22 aa, Homo sapiens
RFLHVPDTFEGHFDGVPVISKG

SEQ ID NO: 325 - protein, 11 aa, Homo sapiens
KYIFHNFMERL

SEQ ID NO: 326 - protein, 35 aa, Homo sapiens
RSFAAGIQALGGTNINDAMLMAVQLLDSSNQEERL

SEQ ID NO: 327 - protein, 18 aa, Homo sapiens
RNMEQFQVSVSVAPNAKI

SEQ ID NO: 328 - protein, 12 aa, Homo sapiens
RVQGNDHSATRE

SEQ ID NO: 329 - protein, 15 aa, Homo sapiens
KWKETLFSVMPGLKM

SEQ ID NO: 330 - protein, 13 aa, Homo sapiens
KAGFSWIEVTFKN

SEQ ID NO: 331 - protein, 31 aa, Homo sapiens
RDQFNLIVFSTEATQWRPSLVPASAENVNKA

SEQ ID NO: 332 - protein, 28 aa, Homo sapiens
RLWAYLTIQQLLEQTVSASDADQQALRN

SEQ ID NO: 333 - protein, 17 aa, Homo sapiens
KFSISGSYVLDQILPRL

SEQ ID NO: 334 - protein, 15 aa, Homo sapiens
KAATGECTATVGKRS

SEQ ID NO: 335 - protein, 13 aa, Homo sapiens
KENFLFLTPDCKS

SEQ ID NO: 336 - protein, 21 aa, Homo sapiens
RDIPTNSPELEETLTHTITKL

SEQ ID NO: 337 - protein, 19 aa, Homo sapiens
KIYPTVNCQPLGMISLMKR

SEQ ID NO: 338 - protein, 15 aa, Homo sapiens
RIGEIKEETTSHLRS

SEQ ID NO: 339 - protein, 17 aa, Homo sapiens
KYNSQNQSNNQFVLYRI

SEQ ID NO: 340 - protein, 13 aa, Homo sapiens
KTVGSDTFYSFKY

SEQ ID NO: 341 - protein, 23 aa, Homo sapiens
RDGFDISGNPWICDQNLSDLYRW

SEQ ID NO: 342 - protein, 25 aa, Homo sapiens
RNALTGLPPGLFQASATLDTLVLKE

SEQ ID NO: 343 - protein, 13 aa, Homo sapiens
KALGHLDLSGNRL

SEQ ID NO: 344 - protein, 12 aa, Homo sapiens
RVAAGAFQGLRQ

SEQ ID NO: 345 - protein, 20 aa, Homo sapiens
RSPVTLLAAVMSLPEEHNKM

SEQ ID NO: 346 - protein, 16 aa, Homo sapiens
KSLEYLDLSFNQIARL

SEQ ID NO: 347 - protein, 20 aa, Homo sapiens
RLTVGAAQVPAQLLVGALRV

SEQ ID NO: 348 - protein, 34 aa, Homo sapiens
REGKEYGVVLAPDGSTVAVEPLLAGLEAGLQGRR

SEQ ID NO: 349 - protein, 17 aa, Homo sapiens
KEFTEAFLGCPAIHPRC

SEQ ID NO: 350 - protein, 15 aa, Homo sapiens
RTDCPGDALFDLLRT

SEQ ID NO: 351 - protein, 17 aa, Homo sapiens
KVAFLTVTLHQGGATRM

SEQ ID NO: 352 - protein, 30 aa, Homo sapiens
RALYYDLISSPDIHGTYKELLDTVTAPQKN

SEQ ID NO: 353 - protein, 12 aa, Homo sapiens
KTVQAVLTVPKL

SEQ ID NO: 354 - protein, 17 aa, Homo sapiens
RLDLQEINNWVQAQMKG

SEQ ID NO: 355 - protein, 15 aa, Homo sapiens
RLVGITSWGEGCARR

SEQ ID NO: 356 - protein, 23 aa, Homo sapiens
KTNLESILSYPKDFTCVHQALKG

SEQ ID NO: 357 - protein, 14 aa, Homo sapiens
RLVLLNAIYLSAKW

SEQ ID NO: 358 - protein, 12 aa, Homo sapiens
KFQPTLLTLPRI

SEQ ID NO: 359 - protein, 13 aa, Homo sapiens
RHSIFTPETNPRA

SEQ ID NO: 360 - protein, 12 aa, Homo sapiens
RFVTWIEGVMRN

SEQ ID NO: 361 - protein, 10 aa, Homo sapiens
RGQIVFMNRE

SEQ ID NO: 362 - protein, 14 aa, Homo sapiens
RDSSTWLTAFVLKV

SEQ ID NO: 363 - protein, 18 aa, Homo sapiens
RYLDKTEQWSTLPPETKD

SEQ ID NO: 364 - protein, 14 aa, Homo sapiens
RDFALLSLQVPLKD

SEQ ID NO: 365 - protein, 25 aa, Homo sapiens
RTLEIPGNSDPNMIPDGDFNSYVRV

SEQ ID NO: 366 - protein, 15 aa, Homo sapiens
REMSGSPASGIPVKV

SEQ ID NO: 367 - protein, 28 aa, Homo sapiens
KLHLETDSLALVALGALDTALYAAGSKS

SEQ ID NO: 368 - protein, 20 aa, Homo sapiens
RGCGEQTMIYLAPTLAASRY

SEQ ID NO: 369 - protein, 15 aa, Homo sapiens
RNELIPLIYLENPRR

SEQ ID NO: 370 - protein, 24 aa, Homo sapiens
KLEAGINQLSFPLSSEPIQGSYRV

SEQ ID NO: 371 - protein, 15 aa, Homo sapiens
RNQGNTWLTAFVLKT

SEQ ID NO: 372 - protein, 19 aa, Homo sapiens
RAFQPFFVELTMPYSVIRG

SEQ ID NO: 373 - protein, 16 aa, Homo sapiens
RIQHPFTVEEFVLPKF

SEQ ID NO: 374 - protein, 14 aa, Homo sapiens
KALLAYAFSLLGKQ

SEQ ID NO: 375 - protein, 11 aa, Homo sapiens
RTLFLLGVTKY

SEQ ID NO: 376 - protein, 13 aa, Homo sapiens
RTVAACNLPIVRG

SEQ ID NO: 377 - protein, 16 aa, Homo sapiens
KWYNLAIGSTCPWLKK

SEQ ID NO: 378 - protein, 12 aa, Homo sapiens
KLILVDYILFKG

SEQ ID NO: 379 - protein, 18 aa, Homo sapiens
RKSPQELLCGASLISDRW

SEQ ID NO: 380 - protein, 15 aa, Homo sapiens
RTATSEYQTFFNPRT

SEQ ID NO: 381 - protein, 19 aa, Homo sapiens
RVTGWGNLKETWTANVGKG

SEQ ID NO: 382 - protein, 22 aa, Homo sapiens
RIVEGSDAEIGMSPWQVMLFRK

SEQ ID NO: 383 - protein, 18 aa, Homo sapiens
KHQDFNSAVQLVENFCRN

SEQ ID NO: 384 - protein, 23 aa, Homo sapiens
RRQECSIPVCGQDQVTVAMTPRS

SEQ ID NO: 385 - protein, 21 aa, Homo sapiens
RLAVTTHGLPCLAWASAQAKA

SEQ ID NO: 386 - protein, 22 aa, Homo sapiens
KGQPSVLQVVNLPIVERPVCKD

SEQ ID NO: 387 - protein, 20 aa, Homo sapiens
RLLNLDGTCADSYSFVFSRD

SEQ ID NO: 388 - protein, 28 aa, Homo sapiens
RLFLGALPGEDSSTSFCLNGLWAQGQRL

SEQ ID NO: 389 - protein, 27 aa, Homo sapiens
RTWDPEGVIFYGDTNPKDDWFMLGLRD

SEQ ID NO: 390 - protein, 16 aa, Homo sapiens
RIALGGLLFPASNLRL

SEQ ID NO: 391 - protein, 26 aa, Homo sapiens
KVVLSSGSGPGLDLPLVLGLPLQLKL

SEQ ID NO: 392 - protein, 10 aa, Homo sapiens
KAVLHIGEKG

SEQ ID NO: 393 - protein, 11 aa, Homo sapiens
KGWVDLFVPKF

SEQ ID NO: 394 - protein, 17 aa, Homo sapiens
KFSISATYDLGATLLKM

SEQ ID NO: 395 - protein, 9 aa, Homo sapiens
RSILFLGKV

SEQ ID NO: 396 - protein, 14 aa, Homo sapiens
RLTLLAPLNSVFKD

SEQ ID NO: 397 - protein, 29 aa, Homo sapiens
KEYANQFMWEYSTNYGQAPLSLLVSYTKS

SEQ ID NO: 398 - protein, 10 aa, Homo sapiens
KELPEHTVKL

SEQ ID NO: 399 - protein, 13 aa, Homo sapiens
RRTHLPEVFLSKV

SEQ ID NO: 400 - protein, 31 aa, Homo sapiens
KTAMDVFVCTYFMPAAQLPELPDVELPTNKD

SEQ ID NO: 401 - protein, 13 aa, Homo sapiens
KLPDATPTELAKL

SEQ ID NO: 402 - protein, 28 aa, Homo sapiens
KELSSFIDKGQELCADYSENTFTEYKKK

SEQ ID NO: 403 - protein, 15 aa, Homo sapiens
KEDFTSLSLVLYSRK

SEQ ID NO: 404 - protein, 25 aa, Homo sapiens
KHQPQEFPTYVEPTNDEICEAFRKD

SEQ ID NO: 405 - protein, 24 aa, Homo sapiens
KHQPQEFPTYVEPTNDEICEAFRK

SEQ ID NO: 406 - protein, 17 aa, Homo sapiens
RKFPSGTFEQVSQLVKE

SEQ ID NO: 407 - protein, 27 aa, Homo sapiens
KELSSFIDKGQELCADYSENTFTEYKK

SEQ ID NO: 408 - protein, 22 aa, Homo sapiens
KEFSHLGKEDFTSLSLVLYSRK

SEQ ID NO: 409 - protein, 23 aa, Homo sapiens
KSYLSMVGSCCTSASPTVCFLKE

SEQ ID NO: 410 - protein, 16 aa, Homo sapiens
RIYISGMAPRPSLAKK

SEQ ID NO: 411 - protein, 20 aa, Homo sapiens
KLIRDVWGIEGPIDAAFTRI

SEQ ID NO: 412 - protein, 20 aa, Homo sapiens
RIGWPNAPILIQDFETLPRE

SEQ ID NO: 413 - protein, 10 aa, Homo sapiens
RLCFFYNKKS

SEQ ID NO: 414 - protein, 10 aa, Homo sapiens
RRPCFESLKA

SEQ ID NO: 415 - protein, 8 aa, Homo sapiens
RIVQIYKD

SEQ ID NO: 416 - protein, 9 aa, Homo sapiens
RFLVNLVKL

SEQ ID NO: 417 - protein, 11 aa, Homo sapiens
KLPNNVLQEKI

SEQ ID NO: 418 - protein, 21 aa, Homo sapiens
RLYGSEAFATDFQDSAAAKKL

SEQ ID NO: 419 - protein, 17 aa, Homo sapiens
KEQLSLLDRFTEDAKRL

SEQ ID NO: 420 - protein, 11 aa, Homo sapiens
REIGELYLPKF

SEQ ID NO: 421 - protein, 10 aa, Homo sapiens
RWRDSLEFRE

SEQ ID NO: 422 - protein, 21 aa, Homo sapiens
KRLYGSEAFATDFQDSAAAKK

SEQ ID NO: 423 - protein, 7 aa, Homo sapiens
RFALVRE

SEQ ID NO: 424 - protein, 10 aa, Homo sapiens
RGVTFLLRRE

SEQ ID NO: 425 - protein, 12 aa, Homo sapiens
RRGEKELLVPRS

SEQ ID NO: 426 - protein, 8 aa, Homo sapiens
KELLVPRS

SEQ ID NO: 427 - protein, 18 aa, Homo sapiens
KNGVAQEPVHLDSPAIKH

SEQ ID NO: 428 - protein, 12 aa, Homo sapiens
RNKFDPSLTQRD

SEQ ID NO: 429 - protein, 20 aa, Homo sapiens
RQLTSGPNQEQVSPLTLLKL

SEQ ID NO: 430 - protein, 11 aa, Homo sapiens
RFMQAVTGWKT

SEQ ID NO: 431 - protein, 16 aa, Homo sapiens
KPKDPTFIPAPIQAKT

SEQ ID NO: 432 - protein, 15 aa, Homo sapiens
RSLDFTELDVAAEKI

SEQ ID NO: 433 - protein, 8 aa, Homo sapiens
RKNLVPRD

SEQ ID NO: 434 - protein, 9 aa, Homo sapiens
RRVWELSKA

SEQ ID NO: 435 - protein, 14 aa, Homo sapiens
KVKIDQTVEELRRS

SEQ ID NO: 436 - protein, 16 aa, Homo sapiens
KDLRDKVNSFFSTFKE

SEQ ID NO: 437 - protein, 13 aa, Homo sapiens
KLVPFATELHERL

SEQ ID NO: 438 - protein, 13 aa, Homo sapiens
RRVEPYGENFNKA

SEQ ID NO: 439 - protein, 11 aa, Homo sapiens
KVNSFFSTFKE

SEQ ID NO: 440 - protein, 17 aa, Homo sapiens
KAVSMPSFSILGSDVRV

SEQ ID NO: 441 - protein, 23 aa, Homo sapiens
KVNWEEEAASGLLTSLKDNVPKA

SEQ ID NO: 442 - protein, 13 aa, Homo sapiens
RDLKVEDIPLARI

SEQ ID NO: 443 - protein, 13 aa, Homo sapiens
KMREWFSETFQKV

SEQ ID NO: 444 - protein, 25 aa, Homo sapiens
KSTAAMSTYTGIFTDQVLSVLKGEE

SEQ ID NO: 445 - protein, 13 aa, Homo sapiens
RAKLEEQAQQIRL

SEQ ID NO: 446 - protein, 8 aa, Homo sapiens
RFWDYLRW

SEQ ID NO: 447 - protein, 16 aa, Homo sapiens
RLKSWFEPLVEDMQRQ

SEQ ID NO: 448 - protein, 8 aa, Homo sapiens
KVSFFCKN

SEQ ID NO: 449 - protein, 16 aa, Homo sapiens
RVCPFAGILENGAVRY

SEQ ID NO: 450 - protein, 24 aa, Homo sapiens
KSNFLNCYVSGFHPSDIEVDLLKN

SEQ ID NO: 451 - protein, 15 aa, Homo sapiens
RLSSGLVTAALYGRL

SEQ ID NO: 452 - protein, 9 aa, Homo sapiens
KIAWHVIRN

SEQ ID NO: 453 - protein, 18 aa, Homo sapiens
KLSNNALSGLPQGVFGKL

SEQ ID NO: 454 - protein, 16 aa, Homo sapiens
RDHLGFQVTWPDESKA

SEQ ID NO: 455 - protein, 8 aa, Homo sapiens
KVYVHLKN

SEQ ID NO: 456 - protein, 21 aa, Homo sapiens
KLISVDTEHSNIYLQNGPDRI

SEQ ID NO: 457 - protein, 28 aa, Homo sapiens
KDVDKEFYLFPTVFDENESLLLEDNIRM

SEQ ID NO: 458 - protein, 13 aa, Homo sapiens
KDIFTGLIGPMKI

SEQ ID NO: 459 - protein, 25 aa, Homo sapiens
RSVPPSASHVAPTETFTYEWTVPKE

SEQ ID NO: 460 - protein, 15 aa, Homo sapiens
KVNKDDEEFIESNKM

SEQ ID NO: 461 - protein, 9 aa, Homo sapiens
RKYNELLKS

SEQ ID NO: 462 - protein, 20 aa, Homo sapiens
RTTLSGAPCQPWASEATYRN

SEQ ID NO: 463 - protein, 23 aa, Homo sapiens
KGHIYQGSEADSVFSGFLIFPSA

SEQ ID NO: 464 - protein, 11 aa, Homo sapiens
KFQSVFTVTRQ

SEQ ID NO: 465 - protein, 14 aa, Homo sapiens
RWILTAAHTLYPKE

SEQ ID NO: 466 - protein, 12 aa, Homo sapiens
KVLNYVDWIKKE

SEQ ID NO: 467 - protein, 10 aa, Homo sapiens
RLPVAPLRKC

SEQ ID NO: 468 - protein, 17 aa, Homo sapiens
RPICLPCTMEANLALRR

SEQ ID NO: 469 - protein, 13 aa, Homo sapiens
RQHLGDVLNFLPL

SEQ ID NO: 470 - protein, 13 aa, Homo sapiens
KLGQYASPTAKRC

SEQ ID NO: 471 - protein, 15 aa, Homo sapiens
KEFPYRIPLDLVPKT

SEQ ID NO: 472 - protein, 9 aa, Homo sapiens
RVFQFLEKS

SEQ ID NO: 473 - protein, 18 aa, Homo sapiens
RMVETTAYALLTSLNLKD

SEQ ID NO: 474 - protein, 17 aa, Homo sapiens
RENSLYLTAFTVIGIRK

SEQ ID NO: 475 - protein, 20 aa, Homo sapiens
KYNPVVIDFEMQPIHEVLRH

SEQ ID NO: 476 - protein, 17 aa, Homo sapiens
KIPGIFELGISSQSDRG

SEQ ID NO: 477 - protein, 14 aa, Homo sapiens
RRPASPISTIQPKA

SEQ ID NO: 478 - protein, 10 aa, Homo sapiens
RFLQEQGHRA

SEQ ID NO: 479 - protein, 10 aa, Homo sapiens
KVSVGGEKRD

SEQ ID NO: 480 - protein, 10 aa, Homo sapiens
KCLVNLIEKV

SEQ ID NO: 481 - protein, 11 aa, Homo sapiens
KKDNEQHVFKV

SEQ ID NO: 482 - protein, 10 aa, Homo sapiens
KISVIRPSKG

SEQ ID NO: 483 - protein, 11 aa, Homo sapiens
KKCLVNLIEKV

SEQ ID NO: 484 - protein, 23 aa, Homo sapiens
RLPPTTTCQQQKEELLPAQDIKA

SEQ ID NO: 485 - protein, 10 aa, Homo sapiens
KLQDEDLGFL

SEQ ID NO: 486 - protein, 13 aa, Homo sapiens
KSCDIPVFMNART

SEQ ID NO: 487 - protein, 12 aa, Homo sapiens
KHGGLYHENMRR

SEQ ID NO: 488 - protein, 10 aa, Homo sapiens
KIIYKENERF

SEQ ID NO: 489 - protein, 16 aa, Homo sapiens
KRAQLGDLPWQVAIKD

SEQ ID NO: 490 - protein, 8 aa, Homo sapiens
KISNLLKF

SEQ ID NO: 491 - protein, 16 aa, Homo sapiens
RRYARTEGNCTALTRG

SEQ ID NO: 492 - protein, 19 aa, Homo sapiens
RVQLGPYQPGRPAACDLRE

SEQ ID NO: 493 - protein, 20 aa, Homo sapiens
RVPEARPNSMVVEHPEFLKA

SEQ ID NO: 494 - protein, 13 aa, Homo sapiens
KAGKEPGLQIWRV

SEQ ID NO: 495 - protein, 22 aa, Homo sapiens
KVWSEVNQAVLDYENRESTPKL

SEQ ID NO: 496 - protein, 18 aa, Homo sapiens
RMLWALLSGPGRRGSTRG

SEQ ID NO: 497 - protein, 8 aa, Homo sapiens
RELISERW

SEQ ID NO: 498 - protein, 14 aa, Homo sapiens
RDVRDYFMPCPGRG

SEQ ID NO: 499 - protein, 14 aa, Homo sapiens
KGDKVWVYPPEKKE

SEQ ID NO: 500 - protein, 13 aa, Homo sapiens
RYYCFQGNQFLRF

SEQ ID NO: 501 - protein, 10 aa, Homo sapiens
RRLWWLDLKS

SEQ ID NO: 502 - protein, 9 aa, Homo sapiens
RLNILNAKF

SEQ ID NO: 503 - protein, 9 aa, Homo sapiens
RNFGYTLRS

SEQ ID NO: 504 - protein, 17 aa, Homo sapiens
KLLPPPPIMSARVLPRP

SEQ ID NO: 505 - protein, 12 aa, Homo sapiens
KRPGVYTQVTKF

SEQ ID NO: 506 - protein, 8 aa, Homo sapiens
KFLNWIKA

SEQ ID NO: 507 - protein, 23 aa, Homo sapiens
MECALDAQSLISISLRKIHSSRT

SEQ ID NO: 508 - protein, 23 aa, Homo sapiens
KAGADTHGRLLQGNICNDAVTKA

SEQ ID NO: 509 - protein, 11 aa, Homo sapiens
KANVFVQLPRL

SEQ ID NO: 510 - protein, 11 aa, Homo sapiens
KELAAQTIKKS

SEQ ID NO: 511 - protein, 15 aa, Homo sapiens
KVTFQLTYEEVLKRN

SEQ ID NO: 512 - protein, 18 aa, Homo sapiens
RTMEQFTIHLTVNPQSKV

SEQ ID NO: 513 - protein, 20 aa, Homo sapiens
RFAHYVVTSQVVNTANEARE

SEQ ID NO: 514 - protein, 22 aa, Homo sapiens
RSSALDMENFRTEVNVLPGAKV

SEQ ID NO: 515 - protein, 11 aa, Homo sapiens
KMKQTVEAMKT

SEQ ID NO: 516 - protein, 9 aa, Homo sapiens
RIYLQPGRL

SEQ ID NO: 517 - protein, 17 aa, Homo sapiens
KHLEVDVWVIEPQGLRF

SEQ ID NO: 518 - protein, 13 aa, Homo sapiens
KFYNQVSTPLLRN

SEQ ID NO: 519 - protein, 10 aa, Homo sapiens
RKLGSYEHRI

SEQ ID NO: 520 - protein, 11 aa, Homo sapiens
KGSEMVVAGKL

SEQ ID NO: 521 - protein, 13 aa, Homo sapiens
RMNFRPGVLSSRQ

SEQ ID NO: 522 - protein, 13 aa, Homo sapiens
KETLFSVMPGLKM

SEQ ID NO: 523 - protein, 12 aa, Homo sapiens
RFKPTLSQQQKS

SEQ ID NO: 524 - protein, 12 aa, Homo sapiens
RRLGVYELLLKV

SEQ ID NO: 525 - protein, 35 aa, Homo sapiens
RDTDRFSSHVGGTLGQFYQEVLWGSPAASDDGRRT

SEQ ID NO: 526 - protein, 10 aa, Homo sapiens
KVRPQQLVKH

SEQ ID NO: 527 - protein, 13 aa, Homo sapiens
RNVHSAGAAGSRM

SEQ ID NO: 528 - protein, 11 aa, Homo sapiens
RLGFTDLFSKW

SEQ ID NO: 529 - protein, 14 aa, Homo sapiens
RVGSALFLSHNLKF

SEQ ID NO: 530 - protein, 10 aa, Homo sapiens
RVQVVAGKKY

SEQ ID NO: 531 - protein, 15 aa, Homo sapiens
RLHLEGNKLQVLGKD

SEQ ID NO: 532 - protein, 10 aa, Homo sapiens
RFNALQYLRL

SEQ ID NO: 533 - protein, 21 aa, Homo sapiens
RIVFENPDPSDGFVLIPDLKW

SEQ ID NO: 534 - protein, 14 aa, Homo sapiens
KILEIEDLFSSLKH

SEQ ID NO: 535 - protein, 8 aa, Homo sapiens
KWFDYLRE

SEQ ID NO: 536 - protein, 34 aa, Homo sapiens
RCELQIRGLAVEDTGEYLCVCGQERTSATLTVRA

SEQ ID NO: 537 - protein, 14 aa, Homo sapiens
KDMKQGLAKLMHRM

SEQ ID NO: 538 - protein, 19 aa, Homo sapiens
KGIVAAFYSGPSLSDKEKL

SEQ ID NO: 539 - protein, 13 aa, Homo sapiens
RTLLLVGSPTWKN

SEQ ID NO: 540 - protein, 16 aa, Homo sapiens
RWYVPVKDLLGIYEKL

SEQ ID NO: 541 - protein, 32 aa, Homo sapiens
RSSTSPTTNVLLSPLSVATALSALSLGAEQRT

SEQ ID NO: 542 - protein, 19 aa, Homo sapiens
KGVTSVSQIFHSPDLAIRD

SEQ ID NO: 543 - protein, 11 aa, Homo sapiens
RDKGQAGLQRA

SEQ ID NO: 544 - protein, 11 aa, Homo sapiens
KSHKPLNMGKV

SEQ ID NO: 545 - protein, 12 aa, Homo sapiens
RFGLLDEDGKKT

SEQ ID NO: 546 - protein, 13 aa, Homo sapiens
KGLCVATPVQLRV

SEQ ID NO: 547 - protein, 11 aa, Homo sapiens
RYRVFALDQKM

SEQ ID NO: 548 - protein, 23 aa, Homo sapiens
KAEFQDALEKLNMGITDLQGLRL

SEQ ID NO: 549 - protein, 34 aa, Homo sapiens
RECVGFEAVQEVPVGLVQPASATLYDYYNPERRC

SEQ ID NO: 550 - protein, 28 aa, Homo sapiens
RVTASDPLDTLGSEGALSPGGVASLLRL

SEQ ID NO: 551 - protein, 16 aa, Homo sapiens
RNELIPLIYLENPRRN

SEQ ID NO: 552 - protein, 13 aa, Homo sapiens
KAVGYLITGYQRQ

SEQ ID NO: 553 - protein, 14 aa, Homo sapiens
RAFIQLWAFDAVKG

SEQ ID NO: 554 - protein, 28 aa, Homo sapiens
RLTEREWADEWKHLDHALNCIMEMVEKT

SEQ ID NO: 555 - protein, 24 aa, Homo sapiens
KALMDLLAGKGSQGSQAPQALDRT

SEQ ID NO: 556 - protein, 19 aa, Homo sapiens
RTFGSGEADCGLRPLFEKK

SEQ ID NO: 557 - protein, 8 aa, Homo sapiens
KISNIIKQ

SEQ ID NO: 558 - protein, 12 aa, Homo sapiens
RFSGTWYAMAKK

SEQ ID NO: 559 - protein, 27 aa, Homo sapiens
RLLNNWDVCADMVGTFTDTEDPAKFKM

SEQ ID NO: 560 - protein, 12 aa, Homo sapiens
KYWGVASFLQKG

SEQ ID NO: 561 - protein, 12 aa, Homo sapiens
RGYVIIKPLVWV

SEQ ID NO: 562 - protein, 14 aa, Homo sapiens
RLPLVPALDGCLRR

SEQ ID NO: 563 - protein, 16 aa, Homo sapiens
RNELIRQEKLEQLARR

SEQ ID NO: 564 - protein, 19 aa, Homo sapiens
KEELATRLNSSETADLLKE

SEQ ID NO: 565 - protein, 16 aa, Homo sapiens
RQCLLNRPFSDNSARD

SEQ ID NO: 566 - protein, 12 aa, Homo sapiens
KNALALFVLPKE

SEQ ID NO: 567 - protein, 11 aa, Homo sapiens
RSFMLLILERS

SEQ ID NO: 568 - protein, 14 aa, Homo sapiens
KTEPKAPEPISSKP

SEQ ID NO: 569 - protein, 15 aa, Homo sapiens
RGSPAINVAVHVFRK

SEQ ID NO: 570 - protein, 28 aa, Homo sapiens
RELISDLEHRLQGSVMELLQGVDGVIKR

SEQ ID NO: 571 - protein, 40 aa, Homo sapiens
KTAMDVFVCTYFMPAAQLPELPDVELPTNKDVCDPGNTKV

SEQ ID NO: 572 - protein, 13 aa, Homo sapiens
KVMDKYTFELSRR

SEQ ID NO: 573 - protein, 28 aa, Homo sapiens
KLAQKVPTADLEDVLPLAEDITNILSKC

SEQ ID NO: 574 - protein, 22 aa, Homo sapiens
KSCESNSPFPVHPGTAECCTKE

SEQ ID NO: 575 - protein, 10 aa, Homo sapiens
RKLCMAALKH

SEQ ID NO: 576 - protein, 10 aa, Homo sapiens
KLCDNLSTKN

SEQ ID NO: 577 - protein, 11 aa, Homo sapiens
RIYISGMAPRP

SEQ ID NO: 578 - protein, 9 aa, Homo sapiens
RERVYFFKG

SEQ ID NO: 579 - protein, 10 aa, Homo sapiens
KAVRPGYPKL

SEQ ID NO: 580 - protein, 8 aa, Homo sapiens
KTRFLLRT

SEQ ID NO: 581 - protein, 30 aa, Homo sapiens
KTYVPPPFSQDLFTFHADMCQSQNEELQRK

SEQ ID NO: 582 - protein, 20 aa, Homo sapiens
KKSDVGFLPPFPTLDPEEKC

SEQ ID NO: 583 - protein, 23 aa, Homo sapiens
RGTHVDLGLASANVDFAFSLYKQ

SEQ ID NO: 584 - protein, 22 aa, Homo sapiens
KSLPAPWLSMAPVSWITPGLKT

SEQ ID NO: 585 - protein, 11 aa, Homo sapiens
RCLAPLEGARF

SEQ ID NO: 586 - protein, 19 aa, Homo sapiens
RWFLLEQPEIQVAHFPFKN

SEQ ID NO: 587 - protein, 13 aa, Homo sapiens
RLCQDLGPGAFRL

SEQ ID NO: 588 - protein, 19 aa, Homo sapiens
RQLKEHAVEGDCDFQLLKL

SEQ ID NO: 589 - protein, 9 aa, Homo sapiens
KCNLLAEKQ

SEQ ID NO: 590 - protein, 18 aa, Homo sapiens
RSLDFTELDVAAEKIDRF

SEQ ID NO: 591 - protein, 14 aa, Homo sapiens
KDPTFIPAPIQAKT

SEQ ID NO: 592 - protein, 27 aa, Homo sapiens
KEPCVESLVSQYFQTVTDYGKDLMEKV

SEQ ID NO: 593 - protein, 20 aa, Homo sapiens
KFSVPAGIVIPSFQALTARF

SEQ ID NO: 594 - protein, 13 aa, Homo sapiens
KEQHLFLPFSYKN

SEQ ID NO: 595 - protein, 18 aa, Homo sapiens
RGIISALLVPPETEEAKQ

SEQ ID NO: 596 - protein, 14 aa, Homo sapiens
KCFKEHSSLAFWKT

SEQ ID NO: 597 - protein, 11 aa, Homo sapiens
KEHSSLAFWKT

SEQ ID NO: 598 - protein, 21 aa, Homo sapiens
RFNKNNEGTYYSPNYNPQSRS

SEQ ID NO: 599 - protein, 22 aa, Homo sapiens
KHYYIGIIETTWDYASDHGEKK

SEQ ID NO: 600 - protein, 11 aa, Homo sapiens
RVVGGLVALRG

SEQ ID NO: 601 - protein, 24 aa, Homo sapiens
KKGHIYQGSEADSVFSGFLIFPSA

SEQ ID NO: 602 - protein, 15 aa, Homo sapiens
RQTHQPPAPNSLIRF

SEQ ID NO: 603 - protein, 21 aa, Homo sapiens
RQFGPYCGHGFPGPLNIETKS

SEQ ID NO: 604 - protein, 33 aa, Homo sapiens
RQPYSYDFPEDVAPALGTSFSHMLGATNPTQKT

SEQ ID NO: 605 - protein, 15 aa, Homo sapiens
RLLGMETMAWQEIRH

SEQ ID NO: 606 - protein, 20 aa, Homo sapiens
RAVGSGATFSHYYYMILSRG

SEQ ID NO: 607 - protein, 16 aa, Homo sapiens
RFGLLDEDGKKTFFRG

SEQ ID NO: 608 - protein, 11 aa, Homo sapiens
KITQVLHFTKD

SEQ ID NO: 609 - protein, 13 aa, Homo sapiens
RIVACASYKPSRE

SEQ ID NO: 610 - protein, 18 aa, Homo sapiens
RSYFPESWLWEVHLVPRR

SEQ ID NO: 611 - protein, 21 aa, Homo sapiens
KQLPGGQNPVSYVYLEVVSKH

SEQ ID NO: 612 - protein, 13 aa, Homo sapiens
KTLLPVSKPEIRS

SEQ ID NO: 613 - protein, 38 aa, Homo sapiens
RGGASEHITTLAYQELPTADLMQEWGDAVQYNPAIIKV

SEQ ID NO: 614 - protein, 14 aa, Homo sapiens
KGTDYHKQPWQAKI

SEQ ID NO: 615 - protein, 13 aa, Homo sapiens
KVKDISEVVTPRF

SEQ ID NO: 616 - protein, 9 aa, Homo sapiens
KQVPAHARD

SEQ ID NO: 617 - protein, 14 aa, Homo sapiens
RGDSGGPLIVHKRS

SEQ ID NO: 618 - protein, 19 aa, Homo sapiens
RFLCTGGVSPYADPNTCRG

SEQ ID NO: 619 - protein, 19 aa, Homo sapiens
KKEAGIPEFYDYDVALIKL

SEQ ID NO: 620 - protein, 13 aa, Homo sapiens
RYGLVTYATYPKI

SEQ ID NO: 621 - protein, 11 aa, Homo sapiens
KEFDHNSNIRY

SEQ ID NO: 622 - protein, 15 aa, Homo sapiens
KWSSPPQCEGLPCKS

SEQ ID NO: 623 - protein, 13 aa, Homo sapiens
RKGEWVALNPLRK

SEQ ID NO: 624 - protein, 12 aa, Homo sapiens
KSLECLHPGTKF

SEQ ID NO: 625 - protein, 17 aa, Homo sapiens
RGLASANVDFAFSLYKH

SEQ ID NO: 626 - protein, 10 aa, Homo sapiens
KLVVLPFPKE

SEQ ID NO: 627 - protein, 20 aa, Homo sapiens
RASSQWVVGPSYFVEYLIKE

SEQ ID NO: 628 - protein, 16 aa, Homo sapiens
RLLGEVDHYQLALGKF

SEQ ID NO: 629 - protein, 19 aa, Homo sapiens
KQTQVSVLPEGGETPLFKQ

SEQ ID NO: 630 - protein, 11 aa, Homo sapiens
KVDGALCMEKS

SEQ ID NO: 631 - protein, 27 aa, Homo sapiens
KSGAQATWTELPWPHEKVDGALCMEKS

SEQ ID NO: 632 - protein, 12 aa, Homo sapiens
RQGHNSVFLIKG

SEQ ID NO: 633 - protein, 11 aa, Homo sapiens
KTLEAQLTPRV

SEQ ID NO: 634 - protein, 16 aa, Homo sapiens
KDSPVLIDFFEDTERY

SEQ ID NO: 635 - protein, 17 aa, Homo sapiens
KALRDFALQNPSAVPRF

SEQ ID NO: 636 - protein, 17 aa, Homo sapiens
RLWLEGNPWDCGCPLKA

SEQ ID NO: 637 - protein, 12 aa, Homo sapiens
RSSALDMENFRT

SEQ ID NO: 638 - protein, 11 aa, Homo sapiens
RSLAPTAAAKR

SEQ ID NO: 639 - protein, 13 aa, Homo sapiens
RLSNENHGIAQRI

SEQ ID NO: 640 - protein, 15 aa, Homo sapiens
RIYGNQDTSSQLKKF

SEQ ID NO: 641 - protein, 24 aa, Homo sapiens
KTGLLLLSDPDKVTIGLLFWDGRG

SEQ ID NO: 642 - protein, 13 aa, Homo sapiens
KIPKPEASFSPRR

SEQ ID NO: 643 - protein, 24 aa, Homo sapiens
RQGPVNLLSDPEQGVEVTGQYERE

SEQ ID NO: 644 - protein, 17 aa, Homo sapiens
RANTVQEATFQMELPKK

SEQ ID NO: 645 - protein, 21 aa, Homo sapiens
RRLDYQEGPPGVEISCWSVEL

SEQ ID NO: 646 - protein, 18 aa, Homo sapiens
KSPEQQETVLDGNLIIRY

SEQ ID NO: 647 - protein, 13 aa, Homo sapiens
KALWEKPFISSRT

SEQ ID NO: 648 - protein, 11 aa, Homo sapiens
RQVVAGLNFRI

SEQ ID NO: 649 - protein, 20 aa, Homo sapiens
KLGQSLDCNAEVYVVPWEKK

SEQ ID NO: 650 - protein, 24 aa, Homo sapiens
RIASFSQNCDIYPGKDFVQPPTKI

SEQ ID NO: 651 - protein, 19 aa, Homo sapiens
RCAGPEAVKGQTLLAVAKS

SEQ ID NO: 652 - protein, 11 aa, Homo sapiens
KGQTLLAVAKS

SEQ ID NO: 653 - protein, 12 aa, Homo sapiens
KDLLLPQPDLRY

SEQ ID NO: 654 - protein, 11 aa, Homo sapiens
KILGPLSYSKI

SEQ ID NO: 655 - protein, 11 aa, Homo sapiens
RQGSFQGGFRS

SEQ ID NO: 656 - protein, 11 aa, Homo sapiens
KYVLPNFEVKI

SEQ ID NO: 657 - protein, 19 aa, Homo sapiens
RLLATLCSAEVCQCAEGKC

SEQ ID NO: 658 - protein, 12 aa, Homo sapiens
RVGDTLNLNLRA

SEQ ID NO: 659 - protein, 16 aa, Homo sapiens
REPFLSCCQFAESLRK

SEQ ID NO: 660 - protein, 15 aa, Homo sapiens
REELVYELNPLDHRG

SEQ ID NO: 661 - protein, 15 aa, Homo sapiens
RGSFEFPVGDAVSKV

SEQ ID NO: 662 - protein, 20 aa, Homo sapiens
KGSFALSFPVESDVAPIARM

SEQ ID NO: 663 - protein, 38 aa, Homo sapiens
RVVAQGVGIPEDSIFTMADRGECVPGEQEPEPILIPRV

SEQ ID NO: 664 - protein, 11 aa, Homo sapiens
RSGIECQLWRS

SEQ ID NO: 665 - protein, 16 aa, Homo sapiens
KMSSINADFAFNLYRR

SEQ ID NO: 666 - protein, 27 aa, Homo sapiens
RMDWLVPATCEPIQSVFFFSGDKYYRV

SEQ ID NO: 667 - protein, 17 aa, Homo sapiens
RDVWGIEGPIDAAFTRI

SEQ ID NO: 668 - protein, 9 aa, Homo sapiens
RSCPDNPKG

SEQ ID NO: 669 - protein, 6 aa, Homo sapiens
LQVLGK

SEQ ID NO: 670 - protein, 14 aa, Homo sapiens
KAAISGENAGLVRA

SEQ ID NO: 671 - protein, 9 aa, Homo sapiens
KVTYDVSRD

SEQ ID NO: 672 - protein, 8 aa, Homo sapiens
KTAGLVRS

SEQ ID NO: 673 - protein, 12 aa, Homo sapiens
RSLAPTAAAKRR

SEQ ID NO: 674 - protein, 9 aa, Homo sapiens
KFQLPGQKL

SEQ ID NO: 675 - protein, 27 aa, Homo sapiens
RDLYHYITSYVVDGEIIIYGPAYSGRE

SEQ ID NO: 676 - protein, 9 aa, Homo sapiens
TLFIFGVTK

SEQ ID NO: 677 - protein, 18 aa, Homo sapiens
NYTYIWWLNGQSLPVSPR

SEQ ID NO: 678 - protein, 8 aa, Homo sapiens
LQLSETNR

SEQ ID NO: 679 - protein, 9 aa, Homo sapiens
ILILPSVTR

SEQ ID NO: 680 - protein, 16 aa, Homo sapiens
KELELQIGNALFIGKH

SEQ ID NO: 681 - protein, 13 aa, Homo sapiens
KAQWANPFDPSKT

SEQ ID NO: 682 - protein, 13 aa, Homo sapiens
KTEDSSSFLIDKT

SEQ ID NO: 683 - protein, 8 aa, Homo sapiens
KFLNDVKT

SEQ ID NO: 684 - protein, 9 aa, Homo sapiens
KLSNAAHKA

SEQ ID NO: 685 - protein, 8 aa, Homo sapiens
RVLDLTRN

SEQ ID NO: 686 - protein, 13 aa, Homo sapiens
KALGHLDLSGNRL

SEQ ID NO: 687 - protein, 15 aa, Homo sapiens
KLPPGLLANFTLLRT

SEQ ID NO: 688 - protein, 20 aa, Homo sapiens
RTLDLGENQLETLPPDLLRG

SEQ ID NO: 689 - protein, 9 aa, Homo sapiens
RGPLQLERL

SEQ ID NO: 690 - protein, 9 aa, Homo sapiens
RLHLEGNKL

SEQ ID NO: 691 - protein, 8 aa, Homo sapiens
KLQVLGKD

SEQ ID NO: 692 - protein, 12 aa, Homo sapiens
KDLLLPQPDLRY

SEQ ID NO: 693 - protein, 12 aa, Homo sapiens
RVAAGAFQGLRQ

SEQ ID NO: 694 - protein, 8 aa, Homo sapiens
RWLQAQKD

SEQ ID NO: 695 - protein, 11 aa, Homo sapiens
KGQTLLAVAKS

SEQ ID NO: 696 - protein, 10 aa, Homo sapiens
RYLFLNGNKL

SEQ ID NO: 697 - protein, 14 aa, Homo sapiens
KHQFLLTGDTQGRY

SEQ ID NO: 698 - protein, 14 aa, Homo sapiens
RSGLSTGWTQLSKL

SEQ ID NO: 699 - protein, 10 aa, Homo sapiens
KLLELTGPKS

SEQ ID NO: 700 - protein, 9 aa, Homo sapiens
RGVTFLLRR

SEQ ID NO: 701 - protein, 8 aa, Homo sapiens
KELLVPRS

SEQ ID NO: 702 - protein, 9 aa, Homo sapiens
RSSTSPDRI

SEQ ID NO: 703 - protein, 17 aa, Homo sapiens
RLELHVDGPPPRPQLRA

SEQ ID NO: 704 - protein, 13 aa, Homo sapiens
RATWSGAVLAGRD

SEQ ID NO: 705 - protein, 24 aa, Homo sapiens
RTPGAAANLELIFVGPQHAGNYRC

SEQ ID NO: 706 - protein, 24 aa, Homo sapiens
RSLALGTFAHTPALASLGLSNNRL

SEQ ID NO: 707 - protein, 10 aa, Homo sapiens
RELVLAGNRL

SEQ ID NO: 708 - protein, 18 aa, Homo sapiens
RLAYLQPALFSGLAELRE

SEQ ID NO: 709 - protein, 8 aa, Homo sapiens
RELDLSRN

SEQ ID NO: 710 - protein, 11 aa, Homo sapiens
KANVFVQLPRL

SEQ ID NO: 711 - protein, 17 aa, Homo sapiens
RNLIAAVAPGAFLGLKA

SEQ ID NO: 712 - protein, 18 aa, Homo sapiens
RVAGLLEDTFPGLLGLRV

SEQ ID NO: 713 - protein, 24 aa, Homo sapiens
RSFEGLGQLEVLTLDHNQLQEVKA

SEQ ID NO: 714 - protein, 10 aa, Homo sapiens
RNLPEQVFRG

SEQ ID NO: 715 - protein, 15 aa, Homo sapiens
RIRPHTFTGLSGLRR

SEQ ID NO: 716 - protein, 10 aa, Homo sapiens
KLEYLLLSRN

SEQ ID NO: 717 - protein, 16 aa, Homo sapiens
RLAELPADALGPLQRA

SEQ ID NO: 718 - protein, 16 aa, Homo sapiens
RLEALPNSLLAPLGRL

SEQ ID NO: 719 - protein, 13 aa, Homo sapiens
RTFTPQPPGLERL

SEQ ID NO: 720 - protein, 14 aa, Homo sapiens
RDFALQNPSAVPRF

SEQ ID NO: 721 - protein, 17 aa, Homo sapiens
KFICPLTGLWPINTLKC

SEQ ID NO: 722 - protein, 16 aa, Homo sapiens
RVCPFAGILENGAVRY

SEQ ID NO: 723 - protein, 8 aa, Homo sapiens
KCTEEGKW

SEQ ID NO: 724 - protein, 27 aa, Homo sapiens
KWSPELPVCAPIICPPPSIPTFATLRV

SEQ ID NO: 725 - protein, 23 aa, Homo sapiens
KATFGCHDGYSLDGPEEIECTKL

SEQ ID NO: 726 - protein, 11 aa, Homo sapiens
KATVVYQGERV

SEQ ID NO: 727 - protein, 8 aa, Homo sapiens
KVSFFCKN

SEQ ID NO: 728 - protein, 20 aa, Homo sapiens
KCSYTEDAQCIDGTIEVPKC

SEQ ID NO: 729 - protein, 11 aa, Homo sapiens
KEHSSLAFWKT

SEQ ID NO: 730 - protein, 10 aa, Homo sapiens
KTDASDVKPC

SEQ ID NO: 731 - protein, 13 aa, Homo sapiens
KSPYQLVLQHSRL

SEQ ID NO: 732 - protein, 9 aa, Homo sapiens
RVLTDELKH

SEQ ID NO: 733 - protein, 25 aa, Homo sapiens
KVISTITNNIQQIIEIEDTFETLRA

SEQ ID NO: 734 - protein, 10 aa, Homo sapiens
KIPSETLNRI

SEQ ID NO: 735 - protein, 11 aa, Homo sapiens
RILGDPEALRD

SEQ ID NO: 736 - protein, 11 aa, Homo sapiens
RDLLNNHILKS

SEQ ID NO: 737 - protein, 8 aa, Homo sapiens
KAIISNKD

SEQ ID NO: 738 - protein, 24 aa, Homo sapiens
KDILATNGVIHYIDELLIPDSAKT

SEQ ID NO: 739 - protein, 21 aa, Homo sapiens
KTLFELAAESDVSTAIDLFRQ

SEQ ID NO: 740 - protein, 15 aa, Homo sapiens
RQAGLGNHLSGSERL

SEQ ID NO: 741 - protein, 14 aa, Homo sapiens
RLTLLAPLNSVFKD

SEQ ID NO: 742 - protein, 13 aa, Homo sapiens
KDGTPPIDAHTRN

SEQ ID NO: 743 - protein, 16 aa, Homo sapiens
KYLYHGQTLETLGGKK

SEQ ID NO: 744 - protein, 17 aa, Homo sapiens
REGVYTVFAPTNEAFRA

SEQ ID NO: 745 - protein, 8 aa, Homo sapiens
RLLGDAKE

SEQ ID NO: 746 - protein, 9 aa, Homo sapiens
KELANILKY

SEQ ID NO: 747 - protein, 20 aa, Homo sapiens
KYHIGDEILVSGGIGALVRL

SEQ ID NO: 748 - protein, 8 aa, Homo sapiens
KLEVSLKN

SEQ ID NO: 749 - protein, 10 aa, Homo sapiens
KNNVVSVNKE

SEQ ID NO: 750 - protein, 15 aa, Homo sapiens
RGDELADSALEIFKQ

SEQ ID NO: 751 - protein, 9 aa, Homo sapiens
KQASAFSRA

SEQ ID NO: 752 - protein, 9 aa, Homo sapiens
RLAPVYQKL

SEQ ID NO: 753 - protein, 21 aa, Homo sapiens
KLISVDTEHSNIYLQNGPDRI

SEQ ID NO: 754 - protein, 14 aa, Homo sapiens
KALYLQYTDETFRT

SEQ ID NO: 755 - protein, 19 aa, Homo sapiens
RTTIEKPVWLGFLGPIIKA

SEQ ID NO: 756 - protein, 8 aa, Homo sapiens
KVYVHLKN

SEQ ID NO: 757 - protein, 12 aa, Homo sapiens
RIYHSHIDAPKD

SEQ ID NO: 758 - protein, 25 aa, Homo sapiens
RHYYIAAEEIIWNYAPSGIDIFTKE

SEQ ID NO: 759 - protein, 8 aa, Homo sapiens
RIGGSYKK

SEQ ID NO: 760 - protein, 12 aa, Homo sapiens
REYTDASFTNRK

SEQ ID NO: 761 - protein, 25 aa, Homo sapiens
RGPEEEHLGILGPVIWAEVGDTIRV

SEQ ID NO: 762 - protein, 8 aa, Homo sapiens
RVTFHNKG

SEQ ID NO: 763 - protein, 15 aa, Homo sapiens
KGAYPLSIEPIGVRF

SEQ ID NO: 764 - protein, 18 aa, Homo sapiens
KNNEGTYYSPNYNPQSRS

SEQ ID NO: 765 - protein, 25 aa, Homo sapiens
RSVPPSASHVAPTETFTYEWTVPKE

SEQ ID NO: 766 - protein, 10 aa, Homo sapiens
KGSLHANGRQ

SEQ ID NO: 767 - protein, 14 aa, Homo sapiens
RQSEDSTFYLGERT

SEQ ID NO: 768 - protein, 19 aa, Homo sapiens
RTYYIAAVEVEWDYSPQRE

SEQ ID NO: 769 - protein, 19 aa, Homo sapiens
KELHHLQEQNVSNAFLDKG

SEQ ID NO: 770 - protein, 10 aa, Homo sapiens
KGEFYIGSKY

SEQ ID NO: 771 - protein, 10 aa, Homo sapiens
RQYTDSTFRV

SEQ ID NO: 772 - protein, 22 aa, Homo sapiens
KAEEEHLGILGPQLHADVGDKV

SEQ ID NO: 773 - protein, 25 aa, Homo sapiens
KLEFALLFLVFDENESWYLDDNIKT

SEQ ID NO: 774 - protein, 10 aa, Homo sapiens
KTYSDHPEKV

SEQ ID NO: 775 - protein, 11 aa, Homo sapiens
RYEYLEGGDRW

SEQ ID NO: 776 - protein, 21 aa, Homo sapiens
RVQLSPDLLATLPEPASPGRQ

SEQ ID NO: 777 - protein, 14 aa, Homo sapiens
RTTDVTQTFGIEKY

SEQ ID NO: 778 - protein, 13 aa, Homo sapiens
REALVPLVADHKC

SEQ ID NO: 779 - protein, 11 aa, Homo sapiens
RLHKPGVYTRV

SEQ ID NO: 780 - protein, 13 aa, Homo sapiens
RVANYVDWINDRI

SEQ ID NO: 781 - protein, 22 aa, Homo sapiens
KFNLTETSEAEIHQSFQHLLRT

SEQ ID NO: 782 - protein, 10 aa, Homo sapiens
KEQLSLLDRF

SEQ ID NO: 783 - protein, 18 aa, Homo sapiens
KYTGNASALFILPDQDKM

SEQ ID NO: 784 - protein, 11 aa, Homo sapiens
REIGELYLPKF

SEQ ID NO: 785 - protein, 22 aa, Homo sapiens
RDYNLNDILLQLGIEEAFTSKA

SEQ ID NO: 786 - protein, 12 aa, Homo sapiens
KADLSGITGARN

SEQ ID NO: 787 - protein, 21 aa, Homo sapiens
KAVLDVFEEGTEASAATAVKI

SEQ ID NO: 788 - protein, 16 aa, Homo sapiens
KLAAAVSNFGYDLYRV

SEQ ID NO: 789 - protein, 19 aa, Homo sapiens
RALYYDLISSPDIHGTYKE

SEQ ID NO: 790 - protein, 13 aa, Homo sapiens
KELLDTVTAPQKN

SEQ ID NO: 791 - protein, 11 aa, Homo sapiens
KSSFVAPLEKS

SEQ ID NO: 792 - protein, 19 aa, Homo sapiens
KEIPDEISILLLGVAHFKG

SEQ ID NO: 793 - protein, 14 aa, Homo sapiens
KTSLEDFYLDEERT

SEQ ID NO: 794 - protein, 24 aa, Homo sapiens
KVTQNLTLIEESLTSEFIHDIDRE

SEQ ID NO: 795 - protein, 12 aa, Homo sapiens
KTVQAVLTVPKL

SEQ ID NO: 796 - protein, 11 aa, Homo sapiens
KLSYEGEVTKS

SEQ ID NO: 797 - protein, 14 aa, Homo sapiens
KLQSLFDSPDFSKI

SEQ ID NO: 798 - protein, 14 aa, Homo sapiens
RDTDTGALLFIGKI

SEQ ID NO: 799 - protein, 12 aa, Homo sapiens
DTDTGALLFIGK

SEQ ID NO: 800 - protein, 10 aa, Homo sapiens
VEHSDLSFSK

SEQ ID NO: 801 - protein, 22 aa, Homo sapiens
ALALPPLGLAPLLNLWAKPQGR

SEQ ID NO: 802 - protein, 5 aa, Homo sapiens
FLYHK

SEQ ID NO: 803 - protein, 14 aa, Homo sapiens
EVFSKPISWEELLQ

SEQ ID NO: 804 - protein, 15 aa, Homo sapiens
FICPLTGLWPINTLK

SEQ ID NO: 805 - protein, 20 aa, Homo sapiens
DVLLLVHNLPQNLTGHIWYK

SEQ ID NO: 806 - protein, 6 aa, Homo sapiens
TLAFVR

SEQ ID NO: 807 - protein, 14 aa, Homo sapiens
ELIEELVNITQNQK

SEQ ID NO: 808 - protein, 9 aa, Homo sapiens
ELPQSIVYK

SEQ ID NO: 809 - protein, 7 aa, Homo sapiens
VVESLAK

SEQ ID NO: 810 - protein, 8 aa, Homo sapiens
YGIEEHGK

SEQ ID NO: 811 - protein, 13 aa, Homo sapiens
LPDTPQGLLGEAR

SEQ ID NO: 812 - protein, 12 aa, Homo sapiens
TNTNEFLIDVDK

SEQ ID NO: 813 - protein, 11 aa, Homo sapiens
AIGLPEELIQK

SEQ ID NO: 814 - protein, 16 aa, Homo sapiens
AEHPTWGDEQLFQTTR

SEQ ID NO: 815 - protein, 11 aa, Homo sapiens
TFLTVYWTPER

SEQ ID NO: 816 - protein, 10 aa, Homo sapiens
SEPRPGVLLR

SEQ ID NO: 817 - protein, 7 aa, Homo sapiens
ALDLSLK

SEQ ID NO: 818 - protein, 13 aa, Homo sapiens
NCSFSIIYPVVIK

SEQ ID NO: 819 - protein, 8 aa, Homo sapiens
IPSNPSHR

SEQ ID NO: 820 - protein, 6 aa, Homo sapiens
TLPFSR

SEQ ID NO: 821 - protein, 22 aa, Homo sapiens
AALAAFNAQNNGSNFQLEEISR

SEQ ID NO: 822 - protein, 19 aa, Homo sapiens
NNQLVAGYLQGPNVNLEEK

SEQ ID NO: 823 - protein, 9 aa, Homo sapiens
EHSSLAFWK

SEQ ID NO: 824 - protein, 11 aa, Homo sapiens
NFPSPVDAAFR

SEQ ID NO: 825 - protein, 14 aa, Homo sapiens
WNFAYWAAHQPWSR

SEQ ID NO: 826 - protein, 10 aa, Homo sapiens
TAVTANLDIR

SEQ ID NO: 827 - protein, 10 aa, Homo sapiens
YNSQLLSFVR

SEQ ID NO: 828 - protein, 25 aa, Homo sapiens
DLYHYITSYVVDGEIIIYGPAYSGR

SEQ ID NO: 829 - protein, 7 aa, Homo sapiens
YQISVNK

SEQ ID NO: 830 - protein, 10 aa, Homo sapiens
LNIGYIEDLK

SEQ ID NO: 831 - protein, 18 aa, Homo sapiens
ENPAVIDFELAPIVDLVR

SEQ ID NO: 832 - protein, 7 aa, Homo sapiens
YYLQGAK

SEQ ID NO: 833 - protein, 9 aa, Homo sapiens
ITGFLKPGK

SEQ ID NO: 834 - protein, 21 aa, Homo sapiens
HELTDEELQSLFTNFANVVDK

SEQ ID NO: 835 - protein, 6 aa, Homo sapiens
FLNWIK

SEQ ID NO: 836 - protein, 8 aa, Homo sapiens
AEIEYLEK

SEQ ID NO: 837 - protein, 7 aa, Homo sapiens
VQEVLLK

SEQ ID NO: 838 - protein, 10 aa, Homo sapiens
TQIDSPLSGK

SEQ ID NO: 839 - protein, 10 aa, Homo sapiens
DFNQFSSGEK

SEQ ID NO: 840 - protein, 8 aa, Homo sapiens
LLELTGPK

SEQ ID NO: 841 - protein, 17 aa, Homo sapiens
NEIVFPAGILQAPFYTR

SEQ ID NO: 842 - protein, 17 aa, Homo sapiens
EFDDDTYDNDIALLQLK

SEQ ID NO: 843 - protein, 13 aa, Homo sapiens
FSLVSGWGQLLDR

SEQ ID NO: 844 - protein, 19 aa, Homo sapiens
LIQDAVTGLTVNGQITGDK

SEQ ID NO: 845 - protein, 10 aa, Homo sapiens
QGHNSVFLIK

SEQ ID NO: 846 - protein, 7 aa, Homo sapiens
ILPSVPK

SEQ ID NO: 847 - protein, 7 aa, Homo sapiens
STLFVPR

SEQ ID NO: 848 - protein, 13 aa, Homo sapiens
GVTGYFTFNLYLK

SEQ ID NO: 849 - protein, 11 aa, Homo sapiens
EALVPLVADHK

SEQ ID NO: 850 - protein, 8 aa, Homo sapiens
SFRPFVPR

SEQ ID NO: 851 - protein, 19 aa, Homo sapiens
GSLVQASEANLQAAQDFVR

SEQ ID NO: 852 - protein, 11 aa, Homo sapiens
ITLPDFTGDLR

SEQ ID NO: 853 - protein, 9 aa, Homo sapiens
DIIKPDPPK

SEQ ID NO: 854 - protein, 13 aa, Homo sapiens
QGFGNVATNTDGK

SEQ ID NO: 855 - protein, 8 aa, Homo sapiens
AVLHIGEK

SEQ ID NO: 856 - protein, 11 aa, Homo sapiens
YENYTSSFFIR

SEQ ID NO: 857 - protein, 19 aa, Homo sapiens
GLQYAAQEGLLALQSELLR

SEQ ID NO: 858 - protein, 14 aa, Homo sapiens
VELAPLPSWQPVGK

SEQ ID NO: 859 - protein, 12 aa, Homo sapiens
CRPINATLAVEK

SEQ ID NO: 860 - protein, 9 aa, Homo sapiens
GIVEECCFR

SEQ ID NO: 861 - protein, 7 aa, Homo sapiens
SILFLGK

SEQ ID NO: 862 - protein, 6 aa, Homo sapiens
HVVQLR

SEQ ID NO: 863 - protein, 10 aa, Homo sapiens
TQILEWAAER

SEQ ID NO: 864 - protein, 9 aa, Homo sapiens
NSDQEIDFK

SEQ ID NO: 865 - protein, 16 aa, Homo sapiens
SGAQATWTELPWPHEK

SEQ ID NO: 866 - protein, 8 aa, Homo sapiens
VRPQQLVK

SEQ ID NO: 867 - protein, 11 aa, Homo sapiens
SEYGAALAWEK

SEQ ID NO: 868 - protein, 8 aa, Homo sapiens
LEEHYELR

SEQ ID NO: 869 - protein, 10 aa, Homo sapiens
IHWESASLLR

SEQ ID NO: 870 - protein, 19 aa, Homo sapiens
NAVVQGLEQPHGLVVHPLR

SEQ ID NO: 871 - protein, 18 aa, Homo sapiens
VTGLDFIPGLHPILTLSK

SEQ ID NO: 872 - protein, 8 aa, Homo sapiens
ALVLELAK

SEQ ID NO: 873 - protein, 11 aa, Homo sapiens
SLQAFVAVAAR

SEQ ID NO: 874 - protein, 10 aa, Homo sapiens
AGFAGDDAPR

SEQ ID NO: 875 - protein, 6 aa, Homo sapiens
YNQLLR

SEQ ID NO: 876 - protein, 11 aa, Homo sapiens
AQETSGEEISK

SEQ ID NO: 877 - protein, 12 aa, Homo sapiens
DSPSVWAAVPGK

SEQ ID NO: 878 - protein, 25 aa, Homo sapiens
ETPEGAEAKPWYEPIYLGGVFQLEK

SEQ ID NO: 879 - protein, 11 aa, Homo sapiens
AVGYLITGYQR

SEQ ID NO: 880 - protein, 10 aa, Homo sapiens
DIPHWLNPTR

SEQ ID NO: 881 - protein, 10 aa, Homo sapiens
QTLSWTVTPK

SEQ ID NO: 882 - protein, 14 aa, Homo sapiens
IQHPFTVEEFVLPK

SEQ ID NO: 883 - protein, 6 aa, Homo sapiens
NEIWYR

SEQ ID NO: 884 - protein, 12 aa, Homo sapiens
AFQVWSDVTPLR

SEQ ID NO: 885 - protein, 8 aa, Homo sapiens
HYINLITR

SEQ ID NO: 886 - protein, 13 aa, Homo sapiens
WWGGQPLWITATK

SEQ ID NO: 887 - protein, 13 aa, Homo sapiens
LDGSTHLNIFFAK

SEQ ID NO: 888 - protein, 11 aa, Homo sapiens
NHYTESISVAK

SEQ ID NO: 889 - protein, 16 aa, Homo sapiens
VSFSSPLVAISGVALR

SEQ ID NO: 890 - protein, 12 aa, Homo sapiens
ALQDQLVLVAAK

SEQ ID NO: 891 - protein, 12 aa, Homo sapiens
DPTFIPAPIQAK

SEQ ID NO: 892 - protein, 6 aa, Homo sapiens
LSETNR

SEQ ID NO: 893 - protein, 8 aa, Homo sapiens
TGAQELLR

SEQ ID NO: 894 - protein, 9 aa, Homo sapiens
IHPSYTNYR

SEQ ID NO: 895 - protein, 22 aa, Homo sapiens
AQPVQVAEGSEPDGFWEALGGK

SEQ ID NO: 896 - protein, 22 aa, Homo sapiens
SFEGLGQLEVLTLDHNQLQEVK

SEQ ID NO: 897 - protein, 7 aa, Homo sapiens
QINSYVK

SEQ ID NO: 898 - protein, 12 aa, Homo sapiens
WILTAAHTLYPK

SEQ ID NO: 899 - protein, 9 aa, Homo sapiens
AKPALEDLR

SEQ ID NO: 900 - protein, 14 aa, Homo sapiens
AVDIPGLEAATPYR

SEQ ID NO: 901 - protein, 10 aa, Homo sapiens
LSITGTYDLK

SEQ ID NO: 902 - protein, 12 aa, Homo sapiens
FLIPNASQAESK

SEQ ID NO: 903 - protein, 9 aa, Homo sapiens
FQSVFTVTR

SEQ ID NO: 904 - protein, 8 aa, Homo sapiens
INPASLDK

SEQ ID NO: 905 - protein, 11 aa, Homo sapiens
IPKPEASFSPR

SEQ ID NO: 906 - protein, 8 aa, Homo sapiens
ITQDAQLK

SEQ ID NO: 907 - protein, 8 aa, Homo sapiens
TSYQVYSK

SEQ ID NO: 908 - protein, 20 aa, Homo sapiens
DVLLLVHNLPQNLPGYFWYK

SEQ ID NO: 909 - protein, 7 aa, Homo sapiens
AGPLQAR

SEQ ID NO: 910 - protein, 8 aa, Homo sapiens
FQLSETNR

SEQ ID NO: 911 - protein, 10 aa, Homo sapiens
LIEIANHVDK

SEQ ID NO: 912 - protein, 7 aa, Homo sapiens
VFQFLEK

SEQ ID NO: 913 - protein, 14 aa, Homo sapiens
VPGLYYFTYHASSR

SEQ ID NO: 914 - protein, 16 aa, Homo sapiens
VSAPSGTGHLPGLNPL

SEQ ID NO: 915 - protein, 7 aa, Homo sapiens
AGITIPR

SEQ ID NO: 916 - protein, 8 aa, Homo sapiens
IRPFFPQQ

SEQ ID NO: 917 - protein, 18 aa, Homo sapiens
SETEIHQGFQHLHQLFAK

SEQ ID NO: 918 - protein, 8 aa, Homo sapiens
TEQAAVAR

SEQ ID NO: 919 - protein, 11 aa, Homo sapiens
TLLPVSKPEIR

SEQ ID NO: 920 - protein, 7 aa, Homo sapiens
YSHYNER

SEQ ID NO: 921 - protein, 19 aa, Homo sapiens
ANDQYLTAAALHNLDEAVK

SEQ ID NO: 922 - protein, 11 aa, Homo sapiens
ATWSGAVLAGR

SEQ ID NO: 923 - protein, 10 aa, Homo sapiens
TYLHTYESEI

SEQ ID NO: 924 - protein, 9 aa, Homo sapiens
YYGYTGAFR

SEQ ID NO: 925 - protein, 7 aa, Homo sapiens
ELANTIK

SEQ ID NO: 926 - protein, 12 aa, Homo sapiens
GEVTYTTSQVSK

SEQ ID NO: 927 - protein, 11 aa, Homo sapiens
LSNENHGIAQR

SEQ ID NO: 928 - protein, 13 aa, Homo sapiens
IRPHTFTGLSGLR

SEQ ID NO: 929 - protein, 10 aa, Homo sapiens
EAQLPVIENK

SEQ ID NO: 930 - protein, 26 aa, Homo sapiens
QRPPDLDTSSNAVDLLFFTDESGDSR

SEQ ID NO: 931 - protein, 7 aa, Homo sapiens
VQTAHFK

SEQ ID NO: 932 - protein, 15 aa, Homo sapiens
ANLINNIFELAGLGK

SEQ ID NO: 933 - protein, 19 aa, Homo sapiens
AHQLAIDTYQEFEETYIPK

SEQ ID NO: 934 - protein, 9 aa, Homo sapiens
DTYVSSFPR

SEQ ID NO: 935 - protein, 18 aa, Homo sapiens
TPSAAYLWVGTGASEAEK

SEQ ID NO: 936 - protein, 14 aa, Homo sapiens
EQLGEFYEALDCLR

SEQ ID NO: 937 - protein, 16 aa, Homo sapiens
SNPVTLNVLYGPDLPR

SEQ ID NO: 938 - protein, 13 aa, Homo sapiens
LWAYLTIQELLAK

SEQ ID NO: 939 - protein, 11 aa, Homo sapiens
VANYVDWINDR

SEQ ID NO: 940 - protein, 22 aa, Homo sapiens
GAVHVVVAETDYQSFAVLYLER

SEQ ID NO: 941 - protein, 25 aa, Homo sapiens
YHFEALADTGISSEFYDNANDLLSK

SEQ ID NO: 942 - protein, 16 aa, Homo sapiens
SCDLALLETYCATPAK

SEQ ID NO: 943 - protein, 12 aa, Homo sapiens
YVVISQGLDKPR

SEQ ID NO: 944 - protein, 10 aa, Homo sapiens
LLDFEFSSGR

SEQ ID NO: 945 - protein, 13 aa, Homo sapiens
TATSEYQTFFNPR

SEQ ID NO: 946 - protein, 11 aa, Homo sapiens
NVNQSLLELHK

SEQ ID NO: 947 - protein, 9 aa, Homo sapiens
LHKPGVYTR

SEQ ID NO: 948 - protein, 10 aa, Homo sapiens
SERPPIFEIR

SEQ ID NO: 949 - protein, 11 aa, Homo sapiens
ALNSIIDVYHK

SEQ ID NO: 950 - protein, 9 aa, Homo sapiens
LSIPQITTK

SEQ ID NO: 951 - protein, 9 aa, Homo sapiens
LFIPQITPK

SEQ ID NO: 952 - protein, 7 aa, Homo sapiens
FIVGFTR

SEQ ID NO: 953 - protein, 23 aa, Homo sapiens
AFLEVNEEGSEAAASTAVVIAGR

SEQ ID NO: 954 - protein, 8 aa, Homo sapiens
FFQYDTWK

SEQ ID NO: 955 - protein, 18 aa, Homo sapiens
GPITSAAELNDPQSILLR

SEQ ID NO: 956 - protein, 14 aa, Homo sapiens
EQSLNVSQDLDTIR

SEQ ID NO: 957 - protein, 13 aa, Homo sapiens
DAVVYPILVEFTR

SEQ ID NO: 958 - protein, 11 aa, Homo sapiens
SGVDLADSNQK

SEQ ID NO: 959 - protein, 23 aa, Homo sapiens
TEFLSNYLTNVDDITLVPGTLGR

SEQ ID NO: 960 - protein, 16 aa, Homo sapiens
TELRPGETLNVNFLLR

SEQ ID NO: 961 - protein, 9 aa, Homo sapiens
YGFYTHVFR

SEQ ID NO: 962 - protein, 13 aa, Homo sapiens
FGFGGSTDSGPIR

SEQ ID NO: 963 - protein, 16 aa, Homo sapiens
TFVNITPAEVGVLVGK

SEQ ID NO: 964 - protein, 14 aa, Homo sapiens
VSEADSSNADWVTK